European Patent Application EP 4 534 683 A1, published April 9, 2025. Title: Novel CRISPR Gene Editing System. Applicant: Institute of Genetics and Developmental Biology, Chinese Academy of Sciences. The sequence listing filed with the application follows.

SEQUENCE LISTING (97 sequences)

SEQ ID NO: 1 - protein, 491 aa, synthetic construct
MITVRKLKLSIMADEELRIQQLKWIKDEQYNQYRALNNGMAFLIADHMLNTAESTKIIYKNNEINKKKKKIYYMEDKIKKENNKLEEEKILKFESDINKLKHEIKILENEKVELELETKNLSEQFKNHYVEDMYTRLDEIPFQYKDNKSLVQNRLKKDFDFYLNNGGKRGERKPTAYKRDYPLLIRGRLLNFYYNKDNVFIKWIAGITFKVELGNKIKNNIELRHTLHQCMNNEKYKVCDSSLQFDNKNNIILNLTIDIPINTSENNFIEGRVMGVDLGMKIPAYASFNDVEYCRAFGDIEDFLRVRTQLQSRMRKLQMALTLIKGGHGRGKKLQALNRLKDKEKDFVNTYNHMISKRIIEYSIKNCCGVINLEYLSLAAREKDLFLTLQPQKSNRIKRNWSYYDLQTKIENKAKKYGIIVKKIDPYLTSQTCHICGNYDEGQRISQEQFECKACNRKFNADYNASKNIALSTKYINNINESEFFKRYKNN

SEQ ID NO: 2 - protein, 603 aa, synthetic construct
MTDVPVSRIRNFSIVAHIDHGKSTLADRLLQDTGTVAARDMKEQFLDNMELERERGITIKLQAARMDYRAKDGNDYVINLIDTPGHVDFSYEVSRSLAACEGALLVVDASQGVEAQTLANVYLALENNLEIVPVLNKIDLPGAEPDRVAGEIEDTIGLDCSEAIHASAKEGIGIREILEAIVQKVPPPADTVDKPLRALIFDSYYDSYRGVIVYFRVMDGRVKKGDKVRLMASGKEYEIDELGVLAPNQCPIDELHAGEVGYLAASIKAVGDARVGDTITLVSKPATEPWPGYTEAKPMVFCGLFPTDSDQFGELREALDRLRLNDAALSYEPETSSAMGFGFRCGFLGLLHMEIVQERLEREYNLDLIATAPSVVYRVTKIDGEVVMIDNPSELPEPQYRETIEEPYVKVEMITPESFVGTLMELSQTRRGVFVDMRYLTQGRTTLIYEIPLAEVVTDFFDQMKSRSRGYASMEYSLIGYRENPLVRLDVLINGDRVDSLSAIVHRDKAYYVGRALVEKLKELIPRHQFKVPIQATIGSRVVASEAIPALRKDVLAKCYGGDISRKKKLLKKQAEGKKRMKAIGTVDVPQSAFMAVLKIDRE

SEQ ID NO: 3 - protein, 439 aa, synthetic construct
MSALSLSRPLAARLARRNIHYAWVVAAVTFLTMLVTAGAVGIPGVLIAPLEAEFGWTNGQISAAFAIRLVLFGLMGPFAAALMNRFGLRPVILASQLLIATGIFGAMAMTQLWQLTLLLGVVVGIGTGLTAMVLGATVVSRWFAARRGLVIGLLTASTATGQLVFLPVLAALTEAVGWRSALALSLVTLMLTAALVMALMRNRPSDLGLPPFGSATPVPEPPRQSLGAMLISPLTTLRDAVRVPMFWLLFGTFFVCGASTNGLVQTHFIALCGDYGMAAVTAAGMLAVIGVFDFFGTVGSGWLSDRYDSRWLLFWYYSLRGLSLVWLPFSDFSFYALSIFAVFYGLDWVATVPPTVKLTAEHFGERSNIVFGWVFTGHQLGAASAAWSAGATRTAYETYLPAFLTAGLLCLAAALVIALFIGSSGLRRRATPGGARAAA

SEQ ID NO: 4 - protein, 411 aa, synthetic construct
MLKAYRYRIYPNKEQEEFFAKTFGACRFVWNKMLEGKLNALNNKEKLPKITPAKYKKQYQFLREVDSLALANVQLNQEKAFRDYFKNKKHFGLPKFKKKKDKQSYTTNNQGNTIRIDFEKQLLYLPKVKTGIKIKLHRIFEGKIKSATITKTKSGNYYVSILVETDKVQNKIKQPKSKICGIDLGLKDFAIITNDNGSCKIENPKYLVRAEKRLKRLQRQLSRKQKGSNNYKKTREKIAKLHEYISNARNDFLHKTSKAIIDENQVIVVEGLSVKALQQSMLSKLVSDVSWGTFLRYLEYKANWYGRELIIVDRFYPSSKTCSVCGYINTQLRLSNRYWECPECNTFHDRDINASKNLYKVGLSRVGTTRTQACGECSDGGTMIYHRSTSQHSMKQEATTSVSGSSSLSSL

SEQ ID NO: 5 - protein, 628 aa, synthetic construct
LSEQLDDTPEQPNEVEETKKRKQRNKGKHPARIWSVFSRYLVSGREHFDKQVLLAHRFRNKLVELELQRRAAANVVIAQASSELQPLIDALAAAEQVLEVSLQELKAVRAKHRRRAESAAQRDAVTNARTARNQASKALSKARKDAFASEAAQVGLWLAEEHHFQAVLAARHAFINDGLYWPTATDVQDRARAMRKGAPPVFRRFGGAEQAGRIAVQIQKSTDKSQSEGGITFEEAFSCSHGFFRLEKKPGRDPLPEIADQPDYKSKRQQLLTYARAWLRVGSEGKGARAKPCWVVADVLLTRQAPKTARIVQVYLDHSVIGDRERWRLSLVLTNQEGWPKPNRASGCMVGIDLGWRLLDTGELRVAYACGADGQHHELRLPASLVKVWRRPDRIQQERDNLFNDVKARLLEWLKGREDLPDWLKEQAEHLHLWKSSTRLSRLVDHWAGRDINWSSQRRIAGDEEILASLRGWVKRNLHLRDYQYHEREQLAAHRLDVYRKWADGLARLYQTAVLEDADWRDLARLPSPEDDAVNETARYNQRMASPGLLASVITNMFAITSRVECANTTRECWRCGHTEAFDAEAQLIRVCPGCGDACDQDESAARVLLARGQALNQSQVAEAAPSS

SEQ ID NO: 6 - protein, 423 aa, synthetic construct
MDDAPRRTIPIKLDVSEERRGDLHQTKSQFLHCANRTSEWAWRYDDYCVTSKSKAENSLYDELREETDLTANLVQKGIRRAIEAVDAGVEKLQQGEQTSQPEFDSWSVVYDKRSASFNDDHATLSTPNGRVTTEYVLPPEDEREDTPFGRYYESDDWDASSATLQYDEQDDTFYLHVTLKNPDYTVDRTERQEASHDDDGAENGVVLGVDLNVTGAFAVTSTGKFIGSADYLTHKRDQYEKRRARLQQTGTRSAHLTIQSIGSRFSDWSLDWLHNRANDLIAEAQATDVDGIIFENLDHIRENIANESKFQQWTYAKFVELVEYKVESTALFVDTVNPAYTSQRCSHCGFTHEDNRDDKEFACQDCGYEVNADYNAAKNIAKRYCGYIHRGQKSRGGWATSQLALESGTLNVNGEYTPSALRG

SEQ ID NO: 7 - protein, 419 aa, synthetic construct
MPIRLSGADYRRAHEACHNAASLWNFFLASIQEYWKENKTDPTEKEMRHFLYEQRPDLRDGLHAHTVQLILSDLMDAISTYRSNRDSGDNNARAPHREKNYRPLEFSAGFGWRVTPDRQHIALSFGKGHKRITLPLPEIADPKTGEILPPERWGSMQLCWNHNARKWSLHVSVPTPKPPQGNPNIIAAIDEGIINPMTVAIETENSYDVLVINGRHARAIKHYRNTRIATLQEKLSRCVKGSKRWHKLNAKRKRIEAMTDSALHNANHQTTRKVADFIQAHDAGRIVAGDVRDIEKNTRKDEAKRIKNTKNQRRRLSQWSRGKQGTLLEHKTGSTVGHINEAWSSKTCPACQTRNHPNGRGYHCHNCGFTCNRDAVGAINILMRAQHGAYTPIDMDKPIRVKYLRATPIFQPKTVPSME

SEQ ID NO: 8 - protein, 617 aa, synthetic construct
MLGFTIPPKRKFQPRLMICKVSEFKANFTSDQIAIIREYQEGLRRLWNFALGQLINADENWHYDKVSKTYVSKCTLVRHQVKDDLSKTWVAHSPVLDRRSRWIVAACQAYPTATTKAGHQRMADKDHVFTRAEVKASGWVGGYGYSCPIQRDHNPGLISNSAMKDSKRGLGILARARDLQDPTIITPDLLKDLDRQLILNVQQKYRMGLLEQLGGAWDKYVKDRYSKESLRRGKPKFKGTNTPVNTIRHPNPNAGGKKPQSADAVRAIGSDVLKIPGFGDVHLPGLDKRWGKSRVKIMQIVEKASGFFVQLTREETPRRVRKVEPRGYAGIDWGWKEENYCSVSWVNEGGETRSQQISKPRFYRESQEQLGKAQQKLDEKLYRRLILWIHHPDTNLLDYVSEGDADILKTCRTVEDLCAHIGVDLNASTIQRLRWKQCGDSQGVKECKQKIKRIHEKTKRRRRSHQYRIASYLTTYSSGIAVEDGLQKKVGKAKAKAKEDGSGFDKNQASAVTGQNKSNRDAAIGQQIDLIDKKTQEFGKSTQRIKFAADLPLSRICCKCLAYDPEMDISKPVYHCTQCGYEGDRDVNSSALIAKIGREPSLQKTIKQKIKKTRKKS

SEQ ID NO: 9 - protein, 494 aa, synthetic construct
MFAIKSMSELVQHHITIQLKAYLSTTQTALFENWTDSLRPLYNLALGLLYEEQQRRWRTNQKFLKNYLDKSSLQTYLNEIENKPDIYPVEWHITKALPECDWLTKEENEVRKKDNTKSLACRTINRDGNFFTPIRPYWHLEEPQKLAKFKCFTNQWLISCNLLTNYHLQKLLNVNMKVRQSFISMNLMEAWKRYQKGDFRKLKFKSKRNPVISLCNKQTNRIKFDPEANNCQLLGKEFGLIEFRGLHNRHQGQIQPRNGSLTKKADGYYLNLVFQVEHKPIPDSDLQVGIDPGLVTLLTLSDGKCISNQRFLKENERHLTVLQKKLSRQTPGSKNWEKTKKALAKIHKQTADHRKYYNHKVSTHLVNKYGAIAIEDTKLTNMNKRPKAEKREDGKGYEHNGAKAKAGLNQSFHDAGLGQLRAFLESKANSYENRHIERVRANYTSQKCSRCGHTDSENRLTQASFHCLKCGLEMPADLNAAINIEQTAFGLDKS

SEQ ID NO: 10 - protein, 664 aa, synthetic construct
MKRVTITIDGEQTKGIVIGTIAANHTAAEWLLTASVSAKSAKVRFDPEEAVAETSSLVMIAPTRTEKYLYLVPDEQVQPVTTIVRKYGLLSPLDWDCPDYPAGDAFEHLFLQNKLWNDLVTIEREHRAKYRELIGSDEETAQMDTEIASIKDRLSVLDEGRKKLRVEHRKKKCPEIDCLDENIKKLKSELKAVASKAKETRAAAKDRIRAAGNDIENLEKDRQAAVIKAYNNSGLWWGNYNAVLESYKKARIKALKDGAELKYHRFDGSGRFTNQIQGGMSVQDLLEGNRNVASLRLVSSGELGDISGKKPPSLDLQSVGSRRDSREYGILAITLYTGTDEQSKKFRRTLSFPVILHRPLPEGATLKSLSVHRKRVGTDFVWSVVFTFTTDCPTYDQRSSTGNRCGLNLGWKKQAGGGLRVATIYDGSDARHITLPQAIIDGLDYVNGDLQGRIDSAANENHAWLLEQWGGDELPESLQELRSMLRRSKRPHPAKFAKAVIAWRNYPEYLGDARDEAEQRRKATKRLTIEMAHKREKLLRRRMDFYRNTAKQLTSVYDVICLDKMDLRRLALLEKGDGTPNELTKIARKQRQQAAISELRECLSKAAAKNGTQIEQVSTASSATCSACKGKMEQVDGIMWRCRECRALVDQDINAAANLFREVL

SEQ ID NO: 11 - protein, 622 aa, synthetic construct
MTSSIEPTSDASKPATTTRVFKYGLLLPRPEDRSAVWEQLRAAHRYYNKLIEIECHRRQAYRELRSELSRQVAVLEGRLAELNAQIDAALAGLQGERKAKRSAKTSGPEKEALKQLKAERKKLSAALKLERAAALNNPVLKTAIEKLDERSHKELLEARANCGVYWGTYLLVEAAVQQARKSKIDPKFKRWNGTGRLGVQVQKGISVSGFFFKAKEQKGGRQLVQVAELDPEAWSSPIRGVRRRLSRTTLRMRINSDAKGKPVWAEWPMVMHRPLPDGAQIMGVTISAHKKADRTFFTVDVACRLPAVVVAPGPRMVGIDLGWRKIGDEIRVASWVDSDGQKGELRLPASIQARIRKARDIRAIRDETRDKMLPVLATLLKPLKTSDEFKERIENLIMWRSFDRLHKLFWFWKNARFAGDEVPWYVFETWHHRDRHLHQYEAGCRSGALGHRREIYRIFAAHVAKHYGKVVLERWDLRKMAERKPPEEDTADSREPNRQRFDAGVSELRLAIVNAVEREGGLIWRTPAALTTMRCHACGHVHDESIVALQHQCVGCSLVWDQDENAGWNLLASGQAMDNDPDLLAAANPPKKPRKPRFTKKKKASPTSSTMEHDEDLSPTGS

SEQ ID NO: 12 - protein, 589 aa, synthetic construct
MIRTYKYSLKAPENFAEDCEDELRRMNDLWNRLIEIDRQRERSFKDLCRSTSAEYAAAQDEIEALREPIDNLYDAIRAERIATRSKEPSDELRARRDELLGRRKALWEICKAIQKAIPKESQAPINEVYKTNVKLARQQSGCFWGNYNAVIESFETAKSKAIKDGGRLHFKSFDGSGRFVNQIQGGMTVTELLAGSHSQAQLTNLVTTNKTKGRFAFTAFTGKDDAGKRFRRQLFSEINYHRPIPADGVIKAVEVVKVPHDGKQKYKWHACFTVALPEVDIKHPKRNIAGVNLGWRQFGGRLRVAVVVDDAGKKTEYFVPAELVSKFEAAETIQKAADDARNEMLSWLRTFYQDNRDEAPQEWRESIQGLLRNRPSVDAANHLMTIWRECVFAQEESRRYAAWLKSDAALRRSYTGCRQNAVKWREEIYRHIAKELAERYAVLAVTDTPLSTMSRTKAKDDLAVDNALPESARRNRVIAAIYSLKEWIGKQAAKTGSTVETITGKMTATCHKCGYVAEKRLRGSQYATCKSCGSELELDENAAINCRNHASGAVLISDKPEKTGRFQRAKMAENDFARKIGDNASPLVT

SEQ ID NO: 13 - protein, 466 aa, synthetic construct
MKTKTIEFKIYPTLAQSQTIDKWLQDIKWVWNKGLSLKFADRQKHYRTQIGDRNIPDGLPLRWKWRKVEATDKKGKITEKWEKIRLVGGGVVRPKSGYPYCPIREHRNIEDPGKFKYFRNDNSPQFVIDIPSEFKEGMADTLKKAWQAYSDPKRPTQKPKFKGKQDKVRSLTSLHAGGKSKLLKPERIPGSDNGFVQFPKLGKLKVKGLYSRHDWVEWGSAKIVKEPSGYYLHVCVDVPNDPLPKSDKSVGIDPGLLSVITTDQGREVAPPKLFRKQQTKLRRLQRKASRQQKGGSNQKKTYQKVALQHEKIRRSRNAFNHKLSTKVVREYSGIVMEDLKIQNLSRKPKAKKREDGNGYEQNGAKRKAGLNKSFADSALGDLISKIETKCKDTDREFVKVAAHHTTVDCSNCGAKIKKALSQRTHRCTECGYEDGRDSNAAKNILIKGQKEFKTVYRAWAWEHGET

SEQ ID NO: 14 - protein, 494 aa, synthetic construct
MFAIKSMSELVQHHITIQLKAYLSTTQTALFENWTDSLRPLYNLALGLLYEEQQRRWRTNQKFLKNYLDKSSLQTYLNEIENKPDIYPVEWHITKALPECDWLTKEENEVRKKDNTKSLACRTINRDGNFFTPIRPYWHLEEPAKLAKFKCFTNQWLISCNLLTNYHLQKLLNVTMKVRQSFISMNLMEAWKRYQKGDFRKLKFKSKRNPVISLCNKQTAIIKFDPEANNCQLLGKEFGLIEFRGLHNRHQGQIQPRNGSLTKKADGYYLNLVFQVEHKPIPDSDLQVGIDPGLVTLLTLSDGKCISNPRFLKENERHLTVLQKKLSRQTPGSKNWEKTKKALAKIHKQTADHRKYYNHKVSTHLVNKYGAIAIEDTKLTNMNKRPKAEKREDGKGYEHNGAKAKAGLNQSLHDAGLGQLRAFLESKANSYENRHIERVKANYTSQKCSRCGHTDKENRLTQASFYCLKCGLEMPADLNAAINIEQAAFGLDKS

SEQ ID NO: 15 - protein, 595 aa, synthetic construct
MVKKPPKEKEDKPKKVIEFKIHPNKEQVEEINRSFASCKLLWNLSIALKEESKQRYYRKNYKFDEFSPEIWELSYSGHYDEEKFKSLKDKEKELLIKNPCCKIAYFKKTSDGKEYTPLNAIPIRRFMNAEDIDKDAVNYLNRQKLAFYFREDTAKFIGEIETEFKKGFFKSVIKTAYDAAKKGIRGIPKFKGRRDKVETLVNGQPDTIKIKSNGVIVSSKIGLLKVRGLDRLQGKAPRMAKITRKATGYYLQLTVETDDTIYKESDKCVGLDMGAVAIFTDDLGRQSEAKRYAKIQKKRLNRLQRQASRQKDNSNNQRKTYAKLARVHEKIARQRKGRNAQLAHKITSEYQSVILEDLKLKNMTAAAKPKEREDGDGYKQNGKKRKSGLNKALLDNAIGQLRTFIENKANERGRKIIRVNPKHTSQTCPNCGNIDKANRVSQSKFKCVSCGYEAHADQNAAANILIRGLQDEFLRAIGSLIKFPVSLIGKYPGLEGKFTPDLDANQESIGDAPIENAEHSISKQMKQEGNRTPTQSENGSQSLIFSSAPPQPCGDSHGKNKPKALPDKASKRSSKKPRGAIPENPDQLTIWDLLD

SEQ ID NO: 16 - protein, 453 aa, synthetic construct
MSKITRKIEIIPDVEGLTHEESNEKCYKAFYNYDRKLYKVANLLVSQLYGLDNLLSLMRLQNEEYVDSQRKLSFKSTTDTAKEEIKKRMEEIDAELMAIKKKIAPMHPQSYSYRAVNSSEYAKDMPSDILDSLKQDVYKHFNDSKKEQIRGERSLTTYKRGMPIPFNLKKKHSIVCDGGNYYLPWFEDTRFRLNFGRDRSNNRAIIDNCIKTKKYKLCAAAKIQLKERKLFLLITVDIPKAESVPVKGKVMGVDLGVVNPAYVAVNDGPERSRIGNGEAFQKQRDVFRRRFRELQRSQLTQGGHGRKHKTKATEILRGKERNWVQTENHRISREIVNLASRWKVETIQMESLKGFGKNQEGEVENNHKRLLGRWSYFELQKDIEYKAAMAGIKVQYVNPAYTSQTCHVCGQRGNRIERDTFICTNPECTCYNQVQDADMNAAINIAKSIKVVK

SEQ ID NO: 17 - protein, 531 aa, synthetic construct
MLQHVGTTWVSWTRTCRAGGGRWVSVASTKTVVLRAFKFTLAPTATQDQQLLRWCGNARLAFNYALASKRAAHTEWRAQVDALVTSGVKEPVARKRVTGPKTPTKPAVYKAFIAERGDTREGLDGVCPWAHEINTHVFQSAFIDADRAWKNWLDSFKGTRKGRRVGYPRFKKRGRARDAFRLHHTVTKPTIRFSTHRRLRLPTFGEVRLHDSARTLVRQIDRGTAVVQSVTVSRAGHRWYASVLCKVEMDLPSGPTRSQQAAGTVGIDFGVKALAALSKPLVPDRPESTLLPNPRHLAKAAHRLKRAQQTLSRRQKGSARREKARRRVARLHHEVAVRRQSALHQITKRLTTRFATIAVEDLHVSGMTRSARGTMDKPGRKVRQKAGLNRAILDASMAEARRQITYKTSWYGSRLAVLDRWWPSSKTCSACGWQNPSLTLADRVFECAQCGLTLDRDLNAARNIEQHAVQVASGTGETQNARGEPVRLPRPRAEKQGSTKREDTGPPGPVPPRRSDPPTPPNPRQGQAKLF

SEQ ID NO: 18 - protein, 470 aa, synthetic construct
MPIITRKIELKIVRLTDEEYDQQWKYLYQINNTIYQAANRISTHCLFNDEYEMRLRLRYMSQCNKIDKKLEKLNPDKKTSDKEEQYRLLNERKELDEDFKNKKQDFQRIKRNSTYQLVSKEFLNYIPAEILTDLNQYVQNNHNNNKNKVKSGERALSTYKKGMGIPFSIKPESGLRLFVKEEGIYLKWFKGILFRLEFGKDASNNRCIVERLIESDKQQKKKGEDYVANNSSIKLVKNGKNTRIFLLLSIDIPAKKQVLDKEVVLGVDLGIKCPLYLAINKDDNFKMQIGDIEHFHNQRTMFQKRFKSLQKLMCTQGGHGRKKKLEPLEKLKEKERNWVHTQNHVYSREVIKQALKQNAGTIHMESLKDFGKGKEGYVKDEYKYLLRYWSYYELQSMIEYKAKLEGIEVKYIDPAYTSQTCSYCGERGERKKQEEFVCTNPQCKRRGEKINADFNAARNIAMSKKIVKDN

SEQ ID NO: 19 - protein, 372 aa, synthetic construct
MINKAYKFRIYPNQAQAILINKTIGCSRFVFNHFLSLWDHAYKETGKGLTYGICSAKLPAMKKELVWLKEVDSIAIQSSVRNLADAYTRFFKNQNSAPRFKSKKNNVQSYTTKQTNENIAVVGNKIKLPKLGLVRFAKSREVEGRIVNATVRRNPSGRYFVSLLVETEVQELPKTHSYIGIDVGLKDFAILSDGTHYENPKFFRSLEEKLAKAQHVLSRRMKGSSRWNKQRVKVARIHEYISNARKDYLDKISTEIIKNHDVIGIEDLQVSNMLKNHKLAKAISEVSWLQFRSMLEYKAKWYGKQVIVVSKTFASSQLCSCCGYQNKDVKNLNLREWFCPSCQTHHDRDINASINLKNEAIRLLTARTAGLA

SEQ ID NO: 20 - protein, 513 aa, synthetic construct
MSSERAPKLRNVVTQQAYKYALEPTPRQQCAFSSHAGAARFAYNWGIARVADSLDAYAEQKAAGIDEPDVKFPGHFDLCKMWTAWKNTAEWTDRHTGQTTTGVPWVASNFVGTYQAALRDAAGAWQRFFRARKTGARAGRPRFKKRGRARDSFQLHGDGLRIVDAKHVNLPKIGTVKTFEATRKLARRLAKGSVPCPTCRATGKITDSASGKVKKCSDCKAAGSRPAARIVRGTVARDSAGRWYLALTVELVREVRTAPTPRQLAGGPVGVDFGVRQVATLSTGQLVDNPRHLESHLRRVKTAQQALSRCPPGSRRRAKAQQRLGRLHARVRHLRENSLQQATSALIHQHSVIAVEGWDVQQTAQHASPKNLPKQIRRNRNRALLDTGIGAARWQLQSKGAWYGTTVVVTDRHAPTGRQCSACGTVKATPIPPTQDEYRCPACGTSLDRRTNTARVLAAVAAQHHDAPSGGESKNARGENTRPTAPRRNGQFSAKREPRSRPPGRGQTGTPGT

SEQ ID NO: 21 - protein, 1227 aa, synthetic construct
MDAKEFTGQYPLSKTLRFELRPIGRTWDNLEASGYLAEDRHRAECYPRAKELLDDNHRAFLNRVLPQIDMDWHPIAEAFCKVHKNPGNKELAQDYNLQLSKRRKEISAYLQDADGYKGLFAKPALDEAMKIAKENGNESDIEVLEAFNGFSVYFTGYHESRENIYSDEDMVSVAYRITEDNFPRFVSNALIFDKLNESHPDIISEVSGNLGVDDIGKYFDVSNYNNFLSQAGIDDYNHIIGGHTTEDGLIQAFNVVLNLRHQKDPGFEKIQFKQLYKQILSVRTSKSYIPKQFDNSKEMVDCICDYVSKIEKSETVERALKLVRNISSFDLRGIFVNKKNLRILSNKLIGDWDAIETALMHSSSSENDKKSVYDSAEAFTLDDIFSSVKKFSDASAEDIGNRAEDICRVISETAPFINDLRAVDLDSLNDDGYEAAVSKIRESLEPYMDLFHELEIFSVGDEFPKCAAFYSELEEVSEQLIEIIPLFNKARSFCTRKRYSTDKIKVNLKFPTLADGWDLNKERDNKAAILRKDGKYYLAILDMKKDLSSIRTSDEDESSFEKMEYKLLPSPVKMLPKIFVKSKAAKEKYGLTDRMLECYDKGMHKSGSAFDLGFCHELIDYYKRCIAEYPGWDVFDFKFRETSDYGSMKEFNEDVAGAGYYMSLRKIPCSEVYRLLDEKSIYLFQIYNKDYSENAHGNKNMHTMYWEGLFSPQNLESPVFKLSGGAELFFRKSSIPNDAKTVHPKGSVLVPRNDVNGRRIPDSIYRELTRYFNRGDCRISDEAKSYLDKVKTKKADHDIVKDRRFTVDKMMFHVPIAMNFKAISKPNLNKKVIDGIIDDQDLKIIGIDRGERNLIYVTMVDRKGNILYQDSLNILNGYDYRKALDVREYDNKEARRNWTKVEGIRKMKEGYLSLAVSKLADMIIENNAIIVMEDLNHGFKAGRSKIEKQVYQKFESMLINKLGYMVLKDKSIDQSGGALHGYQLANHVTTLASVGKQCGVIFYIPAAFTSKIDPTTGFADLFALSNVKNVASMREFFSKMKSVIYDKAEGKFAFTFDYLDYNVKSECGRTLWTVYTVGERFTYSRVNREYVRKVPTDIIYDALQKAGISVEGDLRDRIAESDGDTLKSIFYAFKYALDMRVENREEDYIQSPVKNASGEFFCSKNAGKSLPQDSDANGAYNIALKGILQLRMLSEQYDPNAESIRLPLITNKAWLTFMQSGMKTWKN

SEQ ID NO: 22 - protein, 449 aa, synthetic construct
MTGGNSMGGKVLCQTIRLELEYLYDEDGKRLPYYTELKRIQEQVYLADNRTIQILWEWDNYSVFYKKEHGVAPKAIDFSNGQGSIRGYVYDILKTEFPDWYSGNLTTSIQQTLASYKEVRKDVQAGKRSITSYKKDAPMDIHNACISFEFEGGNAAVSLKVFSEPFRKACGYGSTTVTFKVKKLGKAVREIIELCARGTNGYAFGASKLIYNAKKDCWFLHLAYKFRARENENLDPNHIMGVDLGIKYAAYMGFNHSPERYYIKGGEVETFRHKVEARKRSLQEQGKYCGDGRIGHGYQTRMKPVQKLSDSIARFRDTANHKYSRYIVDMAVKHGCGKIQVEDLSNIKDRQDKFLQEWTYFDLQQKIKYKAEAEGIEVVKVAPHHTSQRCSQCGYIDENNRPSQSEFKCGRCGFTANADYNASLNLATAGIEELIAEELRAKRKNASKH

SEQ ID NO: 23 - protein, 358 aa, synthetic construct
MSQTITVKIKLLSTKEQASILKNMSKEYISTINSLVSEMVAEKKSTKKTTKDVPANLPSAVKNQVIKDAKSVFQKAKKSKYTAVSVLKKPVCIWNNQNYSFDFTHISMPIMIDGKTTKTPIRALLVDKDNRNFDLLKHKLGTLRITQKSGKWIAQISVTIPTVERTGLKVMGVDLGLKVPAVAVTGDDKVRFFGNGRQNKYVRRMFKSKRKKLGKLKKLNAIRNLDDKEQRWMKDQDHKISRAIVDFAKENKISVIRLEQLANIRQTARTSRKNEKNLHTWSFYRLSQFIEYKANLVGIKVEYVNPAYTSQTCPKCSARNKAQDRKYKCECGFEKHRDLVGAMNIRYAPVIDGNSQSA

SEQ ID NO: 24 - protein, 494 aa, synthetic construct
MPIITRKIELKIVKDGLTDEEYDQQWKYLYQINNTIYQAANRISTHCLFNDEYEMRLKLHMPRYKEIDEGLENIKTELEKLNTKKKASDKEKRDRLLNEQRKLVDERKELDKDVKNKKKDFLQCSKQNSTYQLVSKEFLKYIPAEILTDLNQYVQNNYNNNKRKVKSGERALSTYKKGMGIPFSIKPESGLRLFIKENGIYLKWFKLNNDRKEKEILFRLEFGKDTSNNRCIVERLIESDRQQKKKGEDYIANNSSIKLVKNGKNTRIFLLLSIDIPAKKQMLDKDVVLGVDLGIKCPLYLAINKNDNFNMQIGDIEHFHNQRTMFQKRFKSLQKLMCTQGGHGRKKKLEPLEKLKEKERNWVHTQNHVYSREVIKQALKQNAGTIHMESLKDFGKGKDGYVKDEYKYLLRYWSYYELQSMIEYKAKLEGIEVKYIDPAYTSQTCSYCGERGERKKQEEFVCTNPQCKRCGEKINADFNAARNIAMSKKIVKDN

SEQ ID NO: 25 - protein, 575 aa, synthetic construct
MSVSFSLNAKKIRLENYAMKMRLYPSPTQAEQMDKMFLALRLAYNMTFHEVFQQNPAVCGDPDEDGNVWPSYKKMANKTWRKALIDQNPAIAEAPAAAITTNNGLFLSNGQKAWKTGMHNLPANKADRKDFRFYSLSKPRRSFAVQIPPDCIIPSDTNQKVARIKLPKIDGAIKARGFNRKIWFGPDGKHTYEEALAAHELSNNLTVRVSKDTCGDYFICITFSQGKVKGDKPTWEFYQEVRVSPIPEPIGLDVGIKDIAILNTGTKYENKQFKRDRAATLKKMSRQLSRRWGPANSAFRDYNKNIRAENRALEKAQQDPGSSGVGPEAPVLKSVAQPSRRYLTIQKNRAKLERKIARRRDTYYHQVTAEVAGKSSLLAVETLRVKNMLQNHRLAFALSDAAMSDFISKLKYKARRIQVPLVAIGTFQPSSQTCSVCGSINPAVKNLSIRVWTCPNCGTRHNRDINAAKNILAIAQNMLEKKVPFADEALPDEKPPAAPVKKAARKPRDAVFPDHPDLVIRFSKELTQLNDPRYVIVNKATNQIVDNAQGAGYRSAAKAKNCYKAKLAWSSKTNK

SEQ ID NO: 26 - protein, 548 aa, synthetic construct
MPEIVKERITHHAMKMRLYPSPEQAEKIGRIFRALQLAYNITFHAVFCMDPAVCEEPKADGAVWPSYKKMAKAPWRHALIEKNAAIAEAPAGALMTNEGLFLRDARRAWETGMHNLPINKADRKDFRFYHAGKPRRSFLVQMACGNLVPSPDNPKVAWITVQGVPGKMKARGFDRKIWFGAGGAHTYEEAVAAGEVASNLTVCVSQDSCGDYYISVRFSIGKKGARELYRETRACASPVPIGLDVGIKDIAITSEGTKYPNRRPKQRKSPVLERMSRQLSRRWGPANPSFRDYNKAVRQANRTLDQGPPKPLAQPSRGYLAVQRSRARLERRIARQRESYYHQVTAELVRRASMLAVETLHVKNMMQNHRLAYALGDAAMSDFLEKLRYKAERSHVPLVAVGMFEPTSQRCSVCGAQNEAVKSLAVRRWICPSCGAEHDRDINAARNILTIAQTTGPGEDKAKKDAGPRPKRGPRRPRAEVVFADRPQIVVRFSPELTKLNDPRYLIVDKETGAILDDAQGAGYRSITKAKNCYKAKAAWTKKRQETP

SEQ ID NO: 27 - protein, 379 aa, synthetic construct
MEQMTITAKVQIVATDTDKVLLDETMSAYRDACNYVSDYVFQTHDLKQFSLNKVLYSTLREKFGLKSQMAQSVFKTVIARYKTILENQKEWIKPSFKKPQYDLVWNRDYSLTQNCFSVNTLNGRVKLPYFADGMSKYFDHTIYKFGTAKLINKHGKYYLHIPVTYDVEESNISDICNVVGIDRGINFVVATYDSNHKSGFVSGKAIKQKRANYSKLRKELQMRQTPSSRQRIKAIGGRENRWMQDINHQVSKALVENNPKHTLFVLEDLSGIRNTIERVKTKDRYVSVSWSFYDLEQKLIYKAKQNQSSIIKVDPRYTSQCCPCCGHVEKSNRNKKIHLFTCKNCGYKSNDDRIGAMNLYRMGINYLVDSQVPNTVVTE

SEQ ID NO: 28 - protein, 519 aa, synthetic construct
MAETAVLRAFRFALDATAAQEEGFLRHAGASRWAFNHALGMKVAAHRQWQREVKALVEGGMLEAQARKTVKVPVPTRPTIQKHLNRIKGDSRSPDHPEGAQGPQRPCPWFHEVSTYAFQCAFEDADRAWDNWQASLSGRRAGRKVGYPRFKKKGRTKDSFRICHDAKKPTIRPDGYRRLRIPVLGSVRLHDTAKPLARLVDRGASVKSVTVSRSGARWYASVLVSVLQDLPERPTRRQRQAGTVGVDFGVKTLAALSAPVTLPNLGTLTMVPNPRHLASDTRRLTKAQQTLSRTTKGSARRRKAAQRVGIVHHRIASRRATYLHTLTKQLATGYAVVAVEHLNVAGMTSSARGTVEEPGSKVRQKSGLNRSILDASPAEMRRQLDYKTRWNGSQLAVCDRWFPSSRTCSACGWQKPRLTLAERVFNCGQCGLVIDRDLNAARNIAAHAVLVPHGTAAPGSGEASNARGAATRPATPRGGRQAALKREDTGPPRPVPPQRSDPLTLFTLDVPDQQTAKRP

SEQ ID NO: 29 - protein, 488 aa, synthetic construct
MATEYTCITRKIEVHLHKHGDGEEAEQRRAEEFRIWNEINDNLYKAANRIVSHCFFNDAYEYRLKIQSPRYNEIQKSLRYTKRNKLTDDEIKSLKAERKSLFDEFKKQRQTFLRGGVSEGANPEQNSTYKVVSNEFLDVIPSHILTCLNQNVSSTYKCYSKEVEFGNRTIPNFKKGIPVPFPIKHGNILLLKKREDGSIFVDFPKGLEWDLSFGRDRSNNREIVERILSGQYDAGTSSLQEGKNGKIFLLLVVKIPKQSNALDPNRVVGIDLGINIPLYAALNDNEYGGMSIGSREQFLKMRMRMTAQKRELQRNLHYSTNGGRGRSHKLQALERLEGKERNWVHLQNHIFSKNIIEFAVKNNAGVIQMERLTGFGHDRNDEVDDGFKFILRYWSFFELQSMIEYKAEAAGIEVRYIDPYHTSQTCSFCGHYEKGQRIDQATFICKNPECEKGKGKKRSDGTYIGINADWNAARNIALSDKFVDKKKK

SEQ ID NO: 30 - protein, 493 aa, synthetic construct
MKTTEKNVLMTKCIKVTLNRCVNYNMKEIMNIIREMQYLSSKAYNLATNYLYIWDTNSMNFKNLYEEKIVDKDLLGKSKSAWIENRMNEIMKGFLTNNVAQARQDVINKYNKSKKDGLFIGKVTLPSYKMNGKVVIHNKAYRFSKNEGYFVEIGLFNKEKKEELNCDWIKFKLDKIDSNKKATIYKILNGDYKQGSAQLHINKKGKIEFIISYSFERENSIKLDKNRTLGIDIGIVNIAAMAIWDNNKQEWELTRYSHNLISGNEAIALRQKYYKLGLRNKELEKNINRELHELEEKEYRGLSTNIISGHNLTYKRIMLNSKRIRLSQSCKWCGNSKVGHGRRVRCKQVDKIGNKIERFKDTFNHKYSRYIVDFAVKNNCGIIQMENLKNFNPSEKFLKDWPYFDLQTKIEYKAKEYGIEVIKVNPKYTSKRCSRCGCINELNRDCKKNQSKFKCVNDECNNYENADINAAKNIALPYIDKIIEQCLETNKVV

SEQ ID NO: 31 - protein, 509 aa, synthetic construct
MLRAYRLELEIASERKRRFLHQHFGAARFIYNWALRLVREKGFEFFKQGKGGIGKRILYYWREERDKVAPWHHEINAHTFNGAVLDLGRDLKHHSPSQLRGRSRNRHRSAHFYGIKLQHIGRRSIKLPGSRAGEFRGGVYLKVKKGTGKLYEDIQQGRIRTIKRITVSERAGRYFASVLCEVQEPEPLPCTGRVCGLDVGISSIVTVALSDGRIIKQGNPQWLAKKLRRLRRIQRSLARCKTHFPRDPGFKSLHILRRDGEVLAVFPLMWRRQNGELVPEVGDDVRILAEGVASYALLSRAPDRLEKPYRLTVGGQGSGANIELSTMRIRQGHPVRVVHLSVDRSHTMERRRKTLARAHYRVSVAREDFWHRLSTWLVRNCDVIVVESLSIKGMLRSGRFSRHIADAAWGTFFQMLQYKCERYGRTLLRVERSYPSSKKCSRCGKIRKALSLSERTYRCDQCGLKIDRDENAALNLMKLGLAHLTSPTARLAGSDAGGDTIAGGAAACT

SEQ ID NO: 32 - protein, 400 aa, synthetic construct
MITVRKVKLIVNSEEAEEINRTYKFIRDSIYAQYQGLNRCMGYLLSGYYANGMDIKSDGFKNHMKTIKNSLNIFDDINFGIGIDSKSAITQKVKKDFSTSLKNGLAKGERGATNYKRNFPLMTRGRDVKISYLEDINTFVIRWVNKIEFKVILGQKDNIELSHTLHKIINKEYNLGQCTFEFDKNNKLLLALNINIPDNLISKNKEIIPGRVLGVDLGVKVPAMICLNDNTFIKKSIGSYNEFFKVRSQFKARRERLYKQLESSNGGKGRKHKLKATMQFRDKEKNFARTYNHFLSKNIIEFAKKYKCETINLEELNKKGFDNNLLGKWGYYQLQSMIEYKAERVGIKVKYVDPAFTSQTCSKCGYVDEENRITQDKFECQKCGFTLNADHNAAINIARK

SEQ ID NO: 33 - protein, 375 aa, synthetic construct
MTMFERYVKLPVYTINLRLYPTSSQKETIDTIIHELHKACNIAVYDMFTNLTNTTEREDKESKQKIHFPNINTMIKKDYLEKLREERPSISIIPASALSGNNGVFKRDLSKRLDAQVSEGNQKKKTNGKGVKRPIESSKAPYYSKKHPRRSYTYQETLSKIIFNETNDNVVHLNLNKVGRIKARGMKNYLRILRFDETCNMTFKEYCELHKRTAHLFTIKKDNCGDYFIQICLKNVYKLIKDSDNKKEIGIDVGVTDLMILSDGTKYSNPRFKNGEHGEVQKHREQLHRQLSRREGFANIKFREKYKVDHDTLPSKRYQETKLQAAKLERKVARQRKHHMENMVLDVIRQSSFIGIENLSVKDMMKNVKKNKSET

SEQ ID NO: 34 - protein, 472 aa, synthetic construct
MPIITRKIELKIVKDGLTDEEYDQQWKYLYQINNTIYQAANRISTHCLFNDEYEMRLRLRYMSQCNKIDKKLEKLNPDKKTSDKEEQYRLLNERKELDEDFKNKKQDFQRIKRNSTYQLVSKEFLNYIPAEILTDLNQYVQNNHNNNKKKVKSGERALSTYKKGMGIPFSIKPESGLRLFVKEEGIYLKWFKGILFRLEFGKDASNNRCIVERLIESDKQQKKKGEDYVANNSSIKLVKNGKNTRIFLLLSIDIPAKKQVLDKEVVLGVDLGIKCPLYLAINKDDNFKMQIGDIEHFHNQRTMFQKRFKSLQKLMCTQGGHGRKKKLEPLEKLKEKERNWVHTQNHVYSREVIKQALKQNAGTIHMESLKDFGKGKEGYVKDEYKYLLRYWSYYELQSMIEYKAKLEGIEVKYIDPAYTSQTCSYCGERGERKKQEEFVCTNPQCKRRGEKINADFNAARNIAMSKKIVKDN

SEQ ID NO: 35 - protein, 427 aa, synthetic construct
MTKVVKLPLICEQSDKDGNPIDYKKIYEILFELQRQTREIKNKSIQYCWEFSNFSSDYYKQNHEYPKEKDILSYTLVGFVNDKFKTGNDLYSGNCSTTVRGACGEFKNSKTDFLKGTKSIINYKGNQPLDLHNKTIRFECIGKDYYAYLKLLNRPAFQRNNFSSSEIKFKVLVYDNSSKTIVERCIDNIYKISASKLIYNEKKKCWVLNLSYSFTNNNVCELDENKILGVDLGIHYPICASVNGERKFFKIDGGEIDHTRRKIEVRKKSLLKQGSSCGEGRIGHGIKTRNKPVYNIEDKIACFRDTANHKYSRALINYAVNNNCGIIQMEKLTGITADSDRFLKNWSYFDLQTKIEYKAKEAGITVVYIDPQYTSQRCSKCGYISKENRKVQAKFCCQKCGYEANADYNASQNIGIKDIDKIIKNTK

SEQ ID NO: 36 - protein, 402 aa, synthetic construct
MITVRKLKLTIINDDETKRNEQYKFIRDSQYAQYQGLNLAMSVLTNAYLSSNRDIKSDLFKETQKNLKNSSHIFDDITFGKGTDNKSLINQKVKKDFNSAIKNGLARGERNITNYKRTFPLMTRGTALKFSYKDDCSDEIIIKWVNKIVFKVVIGRKDKNYLELMHTLNKVINGEYKVGQSSIYFDKSNKLILNLTLYIPEKKDDDAINGRTLGVDLGIKYPAYVCLNDDTFIRQHIGESLELSKQREQFRNRRKRLQQQLKNVKGGKGREKKLAALDKVAVCERNFVKTYNHTISKRIIDFAKKNKCEFINLEQLTKDGFDNIILSNWSYYELQNMIKYKADREGIKVRYVNPAYTSQKCSKCGYIDKENRPTQEKFKCIKCGFELNADHNAAINISRLEE

SEQ ID NO: 37 - protein, 388 aa, synthetic construct
MRKLRKSFKTEINPTEEQKIKIRKTIGTCRYIYNFYLTHNKELYDNGKKFMSGKSFSVWLNNEYLPNHPEYSWVKEVSSKSVKHSIECGCTAFTRFFKHQSAFPNYKKKGKSDVKMYFVKNNPKDCICERHRINIPTLGWVRIKEKGYIPTTKDGYIIKSGSVSIKVDKFYVSVLVEIPDGQIANNSNDGIGIDLGLKDFAIVSNGKTYKNINKSARLKKLEKQLIREQRCLSRKYDENLKKGEVTQRANIQKQKRKVQKLHHKIDNVRTDYINKTIAEIVKTKPSYITIENLNVKGMMKNRHLSKAVASQKFYEFRAKLQSKCNENGIELRVVARWYPSSKMCHRCGCIKRDLKLSDRIYRCECGYVEDRDFNAALNLRDAITYEVA

SEQ ID NO: 38 - DNA, 542 bp, synthetic construct
  source 1..542: mol_type = other DNA
gtaataacttaactatatagaatatgaatgtgatcgacagcaacaagtgagcggacgcaactaatgtaataacttaactatatagaatatgaattatttaacaagttaaggcgattcaacgtctttggttagaggattatatcactcggcaaaagggttaatgtatgtcaatatgttaccgacatactattctaaaaaataattttgcagtaaatcaaattttcattaaatatgccttaaagttagttgcatcaatatattacatgtatttttaattttgttaataaaatattactatagaattactgcaaaaactttcgttttaaagatgaataatagcactataactatatttacattaggcattcaaagatttttatatacgaactgatttataaattagaaatttagctatataaaaggagtacttaatttaataaggaacaattaaatttttactaatattgagtagttaaatactactctttttttatgctcaattatagaaaggacgtgattatttggatacggaattatggaag

SEQ ID NO: 39 - DNA, 2234 bp, synthetic construct
  source 1..2234: mol_type = other DNA
gtgctcaacgccttacggcatcagaggtttgatcacgtgatcgacagcaacaagtgagcggacgcaactaatgtgctcaacgccttacggcatcagaggtttgatcacagattatctttcggctgattttcgctctctaatgaacgcgaaagatgggcgttttctgaatcgattggtggcatggtgacagatcacaggcgatcggggggtgacgaagcggaggcgaagagcggcggagagtaagccaggtatgaatcggcgggttaaaactccgattttggggagtacgggtttctactgatgcgaaaggatttgaaggaggtggaggcgatcaaaaaggtgaggtggcgaatctgacgacagactcaccacctcacgggattggaaagtttggaatagggctgaaacgagtgctgtgcggtgctgtgcggtgctttgcattttcgtctactcctcaattctgaagcctattctgtaaccttcgtctggaaagtcttgttccaatcgatcgactgcggttggctgtctcttaggtttaatgaaactaatcaggaaagcttgcgacgatcataggttgctgaaatatttgatcgctttgcattcatgctgtttttatgtgcttaacgatacctaaaggcagcaaaatcgagatttttcaagtataaaaacattcatcaaacgccaagatcgatcaaaggtgcaaagactgaaaaattgtatatttgaatacggtttaagataaaattaaagaatttcaaaaacttgtaaaaaaataattcacggtgacttttccaaaaaaattggagtacactacctggggagtgcaggcgtgcaaatacagagcgtcgccgaccgttagcaacgtaaacagtgacagtcatgggaaatagcacaaagtcctcgaaatttccgattgttattgaaatggagccacaggcaaactctgacatcgaagaattggtgaactccggcaaaagtctcatttgtgacaacgtatccgttgccctagagcaactgaaagcccaaggaattttgcccgaaagcgtcatccccgtatttgttgttgttgcatcctccgacgactagtgaagaactgatgtgcaatcatccccaaaggctgctgagctgaagcttaagctgaagttttggggacagatttcgcaagtgtccgatcgtcccgtgtaagcatcagcgcaaatttacccgccgcttgaaacccttacgggacaagcgccgaaatagaaccttacaagcatcttagccgatcgccccgcatctgccaaaacatcacccccgatcgcccttttgccgatcgcccaacccttgccccatctccctttcagccatttacaagcatctccaaagatcccaaaaatcgccaaacccaacccccatcaacattctgcgcccttccagcccctcgccccgccgccaccgccccaggtgcttgtttttgggcaacattcccacccgatcgcccccgcccgatcgcgatccatgccgaaagcccgattgccccattggccccaaacaatccagagcgccaaggcgaattagacgctatggaattcgttacaatgcggttggcttcctttccccgtttgccctaccgttccgctcctggcgatcgacctggggcccatgggagccaaccccttgcaagatggttcaaagcttgagaatttagggtgcattccggcgtaactttcggatcagtgggggttaagggctgttttcagggacttttgcagggcgatcgggactcaccatccccatgcacccggtgaacctcccacagtcgcatccggagttcgttccgcaaagggcgtaaggaacattgagtccttactgggtcacggaacaaagccgatcgaggccgagtgggaaggaagccagtcagcggcgctccgaactacaataggtcatcaaaattcgccaagagcctgatcggtggtctgagtcctactccatccggcatcagtccctgggtaacctgttctgaaaactcgcagtcgccaatgccctaaacccttaccattcgttggctgaagcgatcgaccagttgttcgttgccctttggcatttcaactccccatcatcccgcgctagggcgctatggccggctctttgctcccacaatggatgcttcttcactcccaacggcaacttggcccgcagtttctccagcaccacagcctgggttgcaacccgatcggggctggggggcaagcccc

SEQ ID NO: 40 - DNA, 714 bp, synthetic construct
  source 1..714: mol_type = other DNA
gcttcaatgaggcccgggctgttggcccgggagtcgtgtgatcgacagcaacaagtgagcggacgcaactaatgggcttcaatgaggcccgggctgttggcccgggagtcgtctcgagcgccggatcgccgcgcggttcgatcgcgccggagggggccccacggggtgcccgtccggcgcgggaatccggaccgcgaacgcttagagccctcggcggcgcgcgataagatgtatatacatcgtggccgacatgatgcatatgcatctctgacgttcctctctcctccggcaacaggtcgctccaccggagcgtgacggggctaacggcacggtgtcgcaatgaggcccgggctgttgggctgggagtcgttccggctctatctcgcgctcgccgagaacatgcgattcaagcctcgggaccacctcaagcgcatcgagcacctgaagcttcaatgaggcccgggagtcgtttgactgcaaaagtcaagtctcattccgaatatcagggccccccggatttcccctggccggcgagtgccttgcaggggtgtttgcgaggggtccgcggatgcatgcgggtgcgcatggatttgcccacgttccggttcatccacgataacaaagaacccgccggaatcaaggcgttggccggtctgcgagcgctgggcggaagatctgtcgcgcggcagcgctcgcgccgaggcggcgaagctt

SEQ ID NO: 41 - DNA, 933 bp, synthetic construct
  source 1..933: mol_type = other DNA
ctttcaattccacacggtacattagaaacagtgatcgacagcaacaagtgagcggacgcaactaatctttcaattccacacggtacattagaaacatttcaaaagccataccagagtttagcaggtttgagcgtttctaatgtaccgtgtggaattgaaagtacactcaaacacataaaactttctttttctctttggtttctaatgtaccgtgtggaattgaaagtggtcttccagctccagctccttttcaaaccttacctgtgtttctaatgtaccgtatggaattaaaaggcaaatagggttataataaaagttttaaaaaggaggtaggtgagatgaaagaagtgctttttgctttcaattccacacggtacattagaaacgaggtttttggagctaaatttaaagcatgagtatattctttcaattccacacggtacattagaaaccccaaaagagatattcaagaaaaacattatacatcaacactttgctaaaaggggtacccttttcaaatgaagttaattttcggaaatcttcagttcccaaaaaggggctgaaaaattgccatttctaactattgaaactcaacagttccaaaagtacctcatcaaaacatcaaaacaccaaaatgttttgatgaagacatcaaaggtatactacccctataatcttacaaacacagtccttattcaactgtcaagatgacaaggggcttataaaacccctcaatcctttttttgattttaatccttagagagagaaattgcttatgatatatatcataaagtgtgttgttggttttagctttaacacttccagcaagaagtctggaatcttctaaagtcggagatgaattgcttactgataaaaataggtttcggtatataatatttatgggaatagaaaataaaatcaaggtaaagaaaa

SEQ ID NO: 42 - DNA, 724 bp, synthetic construct
  source 1..724: mol_type = other DNA
gtgacaaagccctgtgcagcgggctcaaagctgcgacgtgatcgacagcaacaagtgagcggacgcaactaatgggtgacaaagccctgtgcagcgggctcaaagctgcgacccgaggagtaatagttctggccaacaagcagtttgagcaccttttggaggaccagtacgatggcgaacagtcgcagcattcagcccgctgcggagggctttggtccagcggtcatcgtagcacgtgctaactctgtcgcccgtcgaaatgagcgctcgcgagtggctgatacaggtctgcgaggcccacagggccaggcagccatggcgtcttgttgattcacaggcaggtccttaaccgcgccaaggctctctgcagcggactaaatgctgcaaaaccaatcggtcccacctttcaggccccctctgttgctaccgtacatccgttcacagagtcagggcctgcgcggcggcgcggtagccgcggctggcgatccggccgacccatgaaggagcgctatctaggctggaacttgcgtcgcttttgagccagaagtggcgctcgcgcgacgcaagttccatactagttagtgtttacggcggctaccgtgtagcaacttgtcgtaacgggtcgtctggttggtaacgcgctcgcgtggctggttgtaacctcttgtcctatcgcgtgctacgctaccgagggacgtgaatcgctcccaaacaggagtcagcg

SEQ ID NO: 43 - DNA, 1132 bp, synthetic construct
  source 1..1132: mol_type = other DNA
catttcatctgaaatccggtgtggtgatcgacagcaacaagtgagcggacgcaacatttcatctgaaatccggtgtgaacgggagtccactgacaagcctcggggcttgaccccgaggcggttgacgtcggatccactgatttaacgtgaggacgctattactaatatgcgaggaaaccggataccctatggttcacatttacaattgttgtctaataaaaatttacgtgtggggaggggagtcggccctgtcagcgagcgtggtgggtttcatcgagtgtcggcttcctccccgacctcaaggatcggggcatccgcctcgtactgcctggcctcgccggggacgtcctcgtcgtctcgacggaccgatcggagtcgaccactgggaccgaacacccccacaccggatttcagatgaaatcgatcgaacgaggggtgggggagagggtggtggcctcggcggtcgaataagaccaaaccggcgcataaacgaattagatggacttagagagattctcgatggtgctgtacctcttactgctacgttactttctgaactctattatatatcttactctagcagtaatctagtagtagtagtgtagtgagagaatccatcttcaggctcctgcaggcacgaagtgatataccgctgcctttctcctggtatctttatattagacgctggctgcctggcgtgagaacgcaacccacgacgcgttcggctcgctcgcgatcgatccgattcgctcacgagcgggtcagttcgctcacagggtacgtcgcgaaaccgatcacccgccgtcctcggtttgcgggccgacaccgggtttcagatgaaatcgatctttcagaccctgacgaactcgatatctatggcctgaggttcttctcccgaatcgttccgcccggtttgcaactacctacctctctcgcttccgtccggtttaggactgttcgaccgcccggatccgacctcctcctcgcagcgctcgtctcccaccctcctcccgtttcgggagagtcgcacccagtgtgccgacggcccatctccagcggtcgggaccactccccggttacccaccactcgtggagggaaagacctaaggaaaattcatctgaaagacggtgt

SEQ ID NO: 44 - DNA, 987 bp, synthetic construct
  source 1..987: mol_type = other DNA
gtgtcgccgatggtggaggtttgggtgatcgacagcaacaagtgagcggacgcaactaatggtgtgtcgccgatggtggaggtttgggcttcctccggccttgtggcgaataagggtgctggtgcgccacctgtccgaatcctggatgtctgatgccgtgccggctgcatgcaatgccgcgcgccaggtctcctggtgcatccggttggtgtcgtcgccacacaggttagcggcaatcgagaggaatgtcactagttcgcgcgaaaaaaatcacaaaatcacgcctgcccttcgcccccgggcacacatctgggaatccaccgtgctcagccttcaagccagccatacagcaccagggaattcccttactaatttctgtgccgaatccttttatcatgcccctcgccaagcgggacagtgctgtgctcagtccgcttggtcatcccctgcgatgtggggtcgccgatggcggatgttaggaatccctataggaatctgtatcctccgttttcggcgacggttttgtagcacaatcatagaccatgtgatagaatgagagtcatgaaaagaagcgccagaaccaaagacagtgagacatggagggttgccgtcgcaattccgcttgtagaggagctgcctctgcttcgggcctgtaacctccacaatcggcgacccatggataacctgttctaggaggttgtgtcctccgttttcggcgacgaaccgtatcatttcgtttgcctgtgccgtgcctgcgccatgcctgcgcgatgcgctgacgggaatcatggggtatacaaaaggggccggtcccgtggagggaaccggccccttgagttcgttcggtgctgccgaatcatttgtggttttcaacgtcgtcggacgctgaaaaccacgtcgaccagcaaactgtagtctcgcggccagcggtctgcggtctgcggtctgcggccacggccagcggcctaccgcgaccgtgccttcgac

SEQ ID NO: 45 - DNA, 541 bp, synthetic construct
  source 1..541: mol_type = other DNA
gtttcaaaatctaatagagattgctgtggattgaaacgtgatcgacagcaacaagtgagcggacgcaactaatgtttcaaaatctaatagagattgctgtggattgaaaccttacgatgttccctggtttcgagggatacggcggtgtagcttcggcagccgcaatctgctggtgagatcaaccagcgatttctaatagagattagttattcatgaaccttgaaaactgaatattcggattgccctctaattcaccgcaatctctattcgcttttggaagaattccgacacagggtagatgttaagttgaagtgattccgagataggctacagccccgatcccgattgacttctaaggactcaactgctcaatcgaccgtcggcccttatgcagtcagggtttcagcgattttggcaggatcaaagtctctcattcagccatctttggggttcagtgtcggaaactgagtgtcaaagctatggctgataaggattctacagcaagcggtaggggcaaaaaatcttgcgaccttaccattaa

SEQ ID NO: 46 - DNA, 858 bp, synthetic construct
  source 1..858: mol_type = other DNA
gtttcaatcccattgctaggattcattaataagaaacgtgatcgacagcaacaagtgagcggacgcaactaatgtttcaatcccattgctaggattcattaataagaaacagcttgatctactaaaccatgtttttccttcaaaagcagtgatcttaatcacatgaacgtcttatttttttagcagttaataatcattttcttttagcgttttgatagctcgtgagctataccttatacccaatcctgtttagataaactgatttacattctatcggttccctgtttcctcttatatttttgctattattaaatcaagagattttgaaccttgaaaactgaataaaaatagatcccctaattttggcgagagccaccgtacccaagtttcaagggggaacgtcggtgaaagaccggaaaagcttgcctttgagtgccatagtgtgctgtcagcaagaagccgcaaggcacagcctgagattacaggctaatccctcctttttaggggatcttcgctaggacttaactatcgctagaacttaactaaaactgacggctcgaagcggggtcaaaatccctggcctcccgtcagatcgccagaaccttgataattaaagagttgtagctgtttcacctctgggttattactaacattgatgtccccaatcactcgcgatcgcgccaagcccatccccataaggattgtgaggttaaatctgacgggactcaaaaaaatggaagcatggggaaatcattttctccctgcttcttgtagggagattcattaggaattttcgtgttcccgtctttgttgacaagaaacaaagatcatttttaattgtcgggggttgcttattct

SEQ ID NO: 47 - DNA, 382 bp, synthetic construct
  source 1..382: mol_type = other DNA
gtctccactacaaagcggcggagcacgcatgtcaacgtgatcgacagcaacaagtgagcggacgcaactaatgtctccactacaaagcggcggagcacgcatgtcaactgcctatcaactatatccttaaaattacgagattattccggggtgatttcgagcacccctttcaattcgtctatttcagaccacggatttgcagttaactctcgttatcatacaagaactcgctccttaaattaaacggttcgagcggtaccgatggtttacgcaggctctcccttgagaaaaatctttgtcacgtgaccacgaatattaatacaacaccgttgtgtaaacacgcaaccatctaatggttattgaataattcgcatacactaaa

SEQ ID NO: 48 - DNA, 350 bp, synthetic construct
  source 1..350: mol_type = other DNA
gtctcagaacccaaagatctgagcttctcttgtgaggtgatcgacagcaacaagtgagcggacgcaactaatgtctcagaacccaaagatctgagcttctcttgtgagatcgctacgctagcaactagctcactttacgtcaagagctactaacacactttacgaacaggtgttaggttcaacgaataccagcttgccaggcttgagcgatctttaccgcacgaggtatcttggcttcttcatctccgggaacagaggtcgtatgcggttgtcaaagagcgcgcggaccggcccttcgtcggtctaagatcccaaagacctgagcttctattgcaatacgcaggaatcac

SEQ ID NO: 49 - DNA, 569 bp, synthetic construct
  source 1..569: mol_type = other DNA
gtctcattaaccaacccaatgagcagggtttgtaacgtgatcgacagcaacaagtgagcggacgcaactaatgtctcattaaccaacccaatgagcagggtttgtaacaacatgtacattatatgggtgataatagcgaccgatgacgtaattaaatattacagtcctaacaggttggtgaaaaactatatttgagacgctaattttgctcaatcgaaccagcatttagtaggaaatcggcttcatcgtcactaaatatagagtcattcaaagccaaaaaagagtttttcaccaacctgctaagtgtaatattacagcgaatggtgtcttattggcgttttatgcctaacacacacattagcattaaccatagtcgctatatgtgcatcacttttcgggattccgatctatgtaattgccaatgcgtctttcgttggtcgatgaatcttattgccttcctacagcgactttactgtactgaaaggagcacggggatttgtctcattaaccagcccaatgagcagggtttgaactttaaacattcagatttcgctaattgcggggctact

SEQ ID NO: 50 - DNA, 585 bp, synthetic construct
  source 1..585: mol_type = other DNA
gttaggatgcccgcaggatgtcatatagttggcaaggtgatcgacagcaacaagtgagcggacgcaactaatgttaggatgcccgcaggatgtcatatagttggcaagatacaattaatttgtgggtgtactagacctactcctagtggtgaatcggtgctgacaacaccatcacgcgactaggtttaatattttaattttactgtataaagtaccaaaaaactattattaattgtggtaaaatattaaagtcagcccacgaaggaatacgggaatattccgtgtggtttcactgacttatctttctcctgaaatagcaggttactcaatccatgtcaccagagagtaagctgtgtatgactttcattgctagtttccgagggtcgctgttttttggcattttttctttttgttttaattggtaaatcgtctgtaacttggtcatggcaagtaaccgaagttcccggcttgccaactcggaggatgtaatgtagttgggggagaatattcatctcccggtgctatttccgataaatcggtcttagcttcctgatgacattccgtattggaatcagagtcaggctt

SEQ ID NO: 51 - DNA, 859 bp, synthetic construct
  source 1..859: mol_type = other DNA
gtttcaatcccattgctaggattcattaataagaaacgtgatcgacagcaacaagtgagcggacgcaactaatgtttcaatcccattgctaggattcattaataagaaacagcttgatctactaaaccatgtttttccttcaaaagcagtgatcttaatcacatgaacgtcttatttttttagcagttaataatcattttcttttagcgttttgatagctcgtgaggtataccttatacccaatcctgtttagataaactgatttacattctatcggttccctgtttcctcttattgcgatcgcgccaagcccatccccataaggattgtgagcttaaatctgacggggctcaaaaaaatgagtgattggggacatcaatgttagtgataacccagaggtgaaacagctacaactctttaattatcaaggttctggcgatctgacgggaggccagggattttgaccccgcttcgagccgtcagttttagttaagttctagcgatagttaagtcctagcgaagatcccctaaaaaggagggattagcctgtaatctcaggctgtgccttgcggcttcttgctgacagcacactatggcactcaaaggcaagcttttccggtctttcaccgacgttcccccttgaaacttgggtacggtggctctcgccaaaattaggggatctatttttattcagttttcaaggttcaaaatctcttgatttaataatagcaaaaatggaagcatggggaaatcattttctccctgcttcttgtagggagattcattaggagttttcgccttcccgtctttgttgacaagaaacaaagatgatttttaattgtcgggggttacttgttct

SEQ ID NO: 52 - DNA, 704 bp, synthetic construct
  source 1..704: mol_type = other DNA
gtttcaatccctaataaggcttaagcttaattgcttcgtgatcgacagcaacaagtgagcggacgcaactaatgtttcaatccctaataaggcttaagcttaattgcttcattaaacctaattgaacttatactagagctaggcactctttcaatttggtatttatctggtttctttacattcttttttgctttcatggtttcgacctcacataaccactaacacactttatattaacttaaaaataaagcacccatcttcccgaaacccttgatgtaaaaggatttcgggtaaggattgcgccccatcattaaaaattcagttttcaaggttctgctcggttcaaaaaattgtttcagcgatcgccgatcgcgttggttggtctaggtacgcgtaccgacgatcgtcgtgaataagtgcggcgttgctgaacggggggatgatagccgaaagatgcgaaacgggaaaaaagagatcgaatcgatcgcgaaaaatgaatttcaggcgttgcataatagagatatgaatggaggaaatcaaaatgcaatgccctgaatgtaaatggttcttccgaacttacactgtagaaaattcctcaagctccctctctgccaagcaatgctctaaagttgataaatatcaatctaacaaaaactcaaagccttagtatacaagctttacaagcacgagttgttgagagtttt

SEQ ID NO: 53 - DNA, 1478 bp, synthetic construct
  source 1..1478: mol_type = other DNA
ggtgattatcatcttgaaatgaaaggtatatccaacgtgatcgacagcaacaagtgagcggacgcaggtgattatcatcttgaaatgaaaggtatatccaactagttataattgtaaaaagcaaaagtcccaccctggttcgctgtgcaagtgggaagcgtggtgggaactgtcaccgcaaaggtatgtatattttttgaaactgcaaaactttttgcgaataaacttttgtaaagtaccctgttttgaacgaagattacacattgttagtgaaaatttggctcgtttaaccatcaacttcttcagaaggtttagtgttgctgtcagttgatttactgttgattctcctgtagagccttcagactgttacacttccaaagatacagatccttgtgtcaagcagagtgtagtaggccatttgtcggttattttcagttgcagtttgggcagttttgctgcaaaaacactttttatctaaaaaatctgttcataaatagcttattctcatttatttttttgtatttttgcagagcattcgcaataaatgcgtttgtgaataataatttcgatatgaaaatagttgaattaaatattcaaatggggttgttggagacccttatgctgagaatttatgtcactcggtaaataccttaattaattatataacaggcaattgttattaatagggtgattatcatcttgaaatgaaaggtatatccaacgtgatcgacagcaacaagtgagcggacgcaggtgattatcattttgaaatgaaaggtatatttaaccgcacgtaagaccgcatcatcggtggctatcaacttgaactgaaaggtatatccaacttgggggtaacgctgacaatggtgctgcgttggtggttatcatcccaaataagagtattctatgcaaattcataaaagtacaattaatttaatgtatgaagaaagccattttgttaataatgatgttggtgtcgttttgttgcaatatttcagcccaaacgcatctaacttttatgggcattcctattacaggtacaagaaaagctatggtgacaaagctaaaggctaaaggatttactgagaaaatacaagaaaatgatgttggtgttgaattgaaaggaaagtatcttggaaaggatgtcagactgtgtgtttataatagcaatataactaagacagtatatctcatagatatatttttcaaaaaaggttattttatggacttgtacgaacaatatcttgactttcgagaaaagttcaatggtatatacggtaagccaacagaagttcttgacgaatcttttgaagaaacattagagtttgggaaactccctatgtgtgcaacatattatgagagttccaaaggcttgatttctttggagatttcagaagataagcattgtgtggaaatatctttccaagataagcgtaatgcagaaattatgagaaaagaaaaacctcaaaaataaaagt

SEQ ID NO: 54 - DNA, 2445 bp, synthetic construct
  source 1..2445: mol_type = other DNA
tcggtcaccccctgcgcgcccggtccgcacgtgatcgacagcaacaagtgagcggacgcaaccggtcaccccctgcgcgcccggtccgcaccagaccggccgaggccagggccttgctcgcgtgctctccgctggcaagcgagccgggccgctccggggagttgccgccgcagaggacgccgattcgtaaggtctcgatgtcgggcaggagcgtcgtggtcacctgggtctccttctcggatgcggtggtccgtgcgccgggcttggtctcgtgcgagcggggcggggcggggtgctgcgtggctaggccgccggtgaggtcatgcacgtcggccgtcacgactcctcccgcttcagcttgaagaggcgctcctcggccctggtcgtccgagtttcgcgtcgcgtctcggccgggagcggctttttgacgttccggagttcggcctgattccggaggccatcaggggtcacgggcttcccctcggacgcctgtttggcgtccgcgcgcagggcgcggatcgtggggcggatcttcttcttgcgtgccatcgtggtctctctgttcggggtgcccgcccgcccctggatggccgggcggtgaggcccgccccggctgcgggagcgctgggcagccggggcgggagtcgggggtcagtcggcgaaggcgtcagtcccgtggaacgcctccgtggcgagcttgacgaagcggcggtcgtggcggtcgcgggcgttcatcgcccggtagcttccggcccgctcccagaaggcgcggccgtacttggtctgcatgaactcgtggagggacgccttgagagaggactccggggtgtagcccacgcgcagcatgaggctccaggcggtcatccaccggttcgccaggacgtgctgcacggcctcgtcctccggggtgtcctcccagacggcgggcactgactacgacctcttcaccaagagtgtccgcgccgggcagagcaaccttctgccgtaacctccgccccccaggggcgtgatgagggggcccctggctacgccggcgggccttctcaccacgatgtgggccactagcggcagccgccgcacccacacctcaggaacagcgatgtcgagcggtaccgctccacctttgaccgctgacgctccatcgctctatcttcgcgagaacccgtggacctgatcgagcgtcacactcacggtccctgagagcgattaggaggctctcctgatggtgcggcacgaacttccagtcgaagcgtggaaaaagtcgacgtacagcggcgacactcacgggcagtgcatcgagatccaggcgatgccggagggcagcgtcgcggtcggcgactccaaggaccgcagcaggggggccttcgtcttcccggcggcggcgtgggcgaacttcgtaaccgaagcaaaaaacgccccgctcacctgactgttcaacccacgtaccccctgccccgaactgctgcgggcggggggtttgtgcttctggtgttctgtgtcgctggctcggtgactatccggcgtgaatgttcagttttgaattgttgtcgatgccgggccggccggacttccaggccgcagccgtcacctcatgacttctcgggccggaccgtaggaccagggtcgccatgtggatgatcgtcggtcacccctgcgcgcccgggccgcacgtgatcgacagcaacaagtgagcggacgcaatcggtcaccccctgcgcgcccggtccgcacgtgatcgacagcaacaagtgagcggacgcaaccggtcaccccctgcgcgcccggtccgcacacttcctgacctgcggcgttagaacagctttgcctgtccttgacgcgggttggggggtgtcggcggatcgctccgccgaggtggcaccggcccgggagggccggtgtcttcccgcttcgtcgagccctgcttctccgcccgggggcgggggagtctgacgggttctccacgggcgttttgggtctcccccgctgggtggccgtgggcgccagggtgaacttgaacgcgcgcagcacgactgtcttggtgcttgccaccgagacccaccttcctccgcccgcacggcacgtcctcgtccacgacacccacgtggtgccgacgtgttggagcatctagggcatggcactgacaaccgggcccgggcggattgagcgtgcaggtgggatgcccgcttcgcgtcgtccctggcgatgcaacgaggctgttcaagcgctggcaacgtcaatccggccgtccagctaacccgttggagcggaacctgcccaggagggcggagcgcagggcgaagcggtggcagggtcgcgacgtgaagatgatcaagcgctttctggtggcgggtgcggcccttgcgctcctcgcacccgcgtccgcgtcagctactccctccgctgccgccgagggagtcaactggcgcatcaagtgccaggccaagg

SEQ ID NO: 55 - DNA, 833 bp, synthetic construct
  source 1..833: mol_type = other DNA
gttggatataccattcaaaacaatgtgatcgacagcaacaagtgagcggacgcaactaatggtagcgttggatataccattcaaaacaatactgacctccttttttattagtggggactgtaatgacaaaattacaattttatttgaaatggcaaagctttcttgcagattattacatacgttagtcgtttcttgttactaacgtatgcaatgattgattactaacgtatgtgataagcaaccacatgcgttagcaataatagcccttataagtatattaccttataactaaaatcagtaaaaaaagacacgattatcaacccccatgcgcacatcatctcagacggctttatattttgatataccattcaaaacaataataaaaccaacattcggccacatagccgtctgtattcttctgttggatataccataataaaaccaactctgtgccggttgtgctgggtgtaggacttgttggatataccattcaaaacaatgttggatataccattcaaaacaatgataaaaccaaccgttagtttctaagtttattaatttcaatgttttgacgtacttcccgagtatagtttcctatctcaggttaaggacttccagcagccccaattagaaaatttctttttgtaataataggcatactctttttaattttacaaccgcaaatattgtaattataattgtaagtctcaaatccaactcaaataattttcagaatttcacaaattctcaaaatcgcccataaaaaatcccccatgcaaccgcatgagggattccacaagtaaattctatttcgagaaatttattttgctaca

SEQ ID NO: 56 - DNA, 2363 bp, synthetic construct
  source 1..2363: mol_type = other DNA
agttttaatccacgcacccacaagagatacgacgtgatcgacagcaacaagtgagcggacgcaactaattttaatccacgtacctatttgaggtgcgacattcggatgacatggctggtgcagtatatgacttctgatttttttccattcttgttttatgttcctctgctgttggtactaatcgtaaatgtctacagtctttttcattttactatctcctctattttgtaactttttatgattcataaccccgcctacaaacttgaaaacaacacaaaaagagcttcttcaagtcgattgaaaatgtgcatagcaaaataagctatatacactaatcggctcaaagaagccctttcacaattgaaacaagacgaaacttgcttctacaactcaaccacaacacaaaaaaggtgtaggaataaacggaatcaaataaactaacaatatacctttatattacataataacattataggtttcaataagtattaattaaaattaacgcattagccaaaagaattcttattcctcaagcttgtgtaggacgaaagtccaaaggtaagtgagagttgaattttgggtaatgcgtaaactcataataaattgctatcaagggtcttaccagttttaatccacgcacccacaagagatacgacgtgatcgacagcaacaagtgagcggacgcaactaattttaatccacgtacctatttgaggtgcgaccccgatttgtgttcaaaatcaaccacaaatacgttaattctattcaaaagtataaaaatatttttatttagtaaagtaatttttataaaaattataaattcaccccataaagtataagaattctaggtgcgaatgtactaggaatttcatgtttgctatacattcgtacctaaaaaattaaagagatttctaaatcaatttattcttttacaccaatatgttcgaccctattttcatagctattacctaactgattaacaaaaatgtatagtttcataataccctttgtatattgattcataatttacaatgaaattcactatctattgtctctctatctacctatcaagcttaactttcgtatgatcatttaatcttttttaccagataacattcttgaaagcattgaatacgaaatgcaatttctttcgataacttacgaatacttttataattcttatctttatacgtgttcatcctttttagagtaatagtatcagtatgtccaagttttttagatcttttacaccagaaccctctacttcattccataagtaacaggtgcttcttctgactacccatatttttcacttttataattaatttttaactcttcacctattactactctgtgtttcttatatttgtttactatcctctatactattaatttcttccatcttcttattccactatttttattaccgttttccgacatcgttatctatcctttctctattatttatgcgtaaaaagcaggagttaattgctagattcaatattattaccacgctttgtacaaaaatagattactaaaaagaaataaagataaaatgcagattatgtcgaaattagttaaagaatattgaaattcaacatagaatcttatactgaattatcattttatttaataacgaagtcgttcgatacttggtttaaagcctcacggcctgccaagcgagttactgcagcaatagaggctatgcacacatacaaaaaaggatagattcttccaaaaaggaagtatgtcaagatccaaaaaattcattcttgaactacccccactttcacttcgtttagaagtgagggattcctaagtaaagagttctatcgaactctaattaattaggctaaccccgcagtcctttgcttgtgcttgatttggatagatacgaaacttataggctttattaatcattatttgattcacctccattttggtatatgactattatacaccaaacgtacattcgataggtagtggagtaacactttctgtatgtcgaacaattaagatggcttcctgccatcccttgttcgaagccaattcatctcccaccttattcactgggctgtgacccttcacgctccttgaggaaggagtcttcttggctaaaatgataaaatcgtatatagaatgtagtaattaaaaagatcataaagttattcattatctctcttcgtcttaatctctaatatacgcatataaatgagacttcctttgacaaataaagataaaatttattttatctttatcttatctttatctctttatgttagtctgttttcctagaagaaataatcctaatattaaaaagaaacagaggaataatgcatgaagagtaaaaaaatgtttgtatt

SEQ ID NO: 57 - DNA, 925 bp, synthetic construct
  source 1..925: mol_type = other DNA
gacgcctggctcgacacccccaccgaacactggccgctgaccctgccgccggccacgacagacccgcccccgaggtcctagaccgcgagacgagaggacgagttgtcgggccgccgccgcagcggtgatcggtgagcccgacagggaggcgtaagcggccgcgcggtcggcggtgatccgcgcggtgtcataccgcaagcagcttcgacagcacctgcgatccaggctgtagcacgcggagagacgcgcgtagtccatctcggaacgggtccgggccgccgcccgggcgcgctgggagacggtgatcgacagcaacaagtgagcggacgcaactacccgtcgcccgtgtgcgctgggagacggtgatcgacagcaacaagtgagcggacgcaactacccgtcgcccgtgtgcgctgggagacgccccttcccgagctggtgtcttctcccgaccgctgtgaagttgtggggtgcacggacgcccggaccttacgttccgggggtccccgtctgacctcggccgggtggccgggagcggggttctcgtttcgccgagaactgctcagcttcggcgccctctccgacgacatcggcccctccacattccggcaccgtaaggctaccaacgaaaccgaccccgcccgcacagtgcccgaagcagccatgcggccgatgccgggccgtccccgggccgccgggcaggagcacgcgggggccgaggacaccgcgcgccggccggctgccggggcgcagagccggggcgcatgcccgcgcgagccgcgcggcgggaccgccacccggatcgccgaagccgccggcctcggcaccggtccgagcggcgcaggctccggcggccaggtgcttcgctggggcggccgacgggcggccgccccagcgtgacgtcaggtacgcggcttgagcctga

SEQ ID NO: 58 - DNA, 841 bp, synthetic construct
  source 1..841: mol_type = other DNA
tctacactagtagaaattctgaatgagttttagacgtgatcgacagcaacaagtgagcggactctacactagtagaaattctgaatgagttttagacccaggtcccggaccgtaactttaatccgaatgattccgatgtggaagacagcctttcggcctgtttgtgtttggcgacttaaacgaatcgaaaggccgcttttattctatcgccagcagaccgtatcgtgcagggcgtcagcccctgcaccatatcaaaaattcacttgataactgtcacactcgggtcttaatcaatctacactagtagaaattctgaatgagttttagacgtgatcgacagcaacaagtgagcggactctacactagtagaaattctgaatgagttttagacttacctaacataaactgtatgtaagtaatggtatataacacctcttaccgtaccctagccagcatatgaaaaattgatcagaaaacaggattgcgattacttagcacgcgcagaatttgggttttagactggacacggtccaacacggtccaaccatttagacccgatagttcgtacaaggcccattttaatcggtttaacgcgttagatcaatgttatatatcataaataaacgtttttttcatcatatatatacagattcggacatcgtgctgaaaagaagacggaggtttgtccatccatgctaagtaatccgcctgtgtgcatatataattttgtataccaaatgttttatttatttttataacataatattgttattaatgtaattttgcaattatatataagaacgcacatgcagccaacatgaagtccggcggacgcaggaac

SEQ ID NO: 59 - DNA, 1091 bp, synthetic construct
  source 1..1091: mol_type = other DNA
gacgcacaccgcacgcgggtatgggctgagagggtgatcgacagcaacaagtgagcggacgcaactgacgcacaccgcacgcgggtatgggctgagaggttggacaaggcgctggacgtgaccgacctgcactttgcgttggatcccgtgcctgcgcccgatgcgccctgcgcccgcgtgctggacacgacgtatttcacgcttgatctgctgaaggtggatggcgaagcggcggtgcccgcggtgcaggacttcggcattctgacggcgctggacgctgtggagctggcatggcagggcggagctcgccgtctggcggcgggcgagaccgtgctggtaccggccagtgcaccggagatgacggtgaaggggcagggaagagtggcgctgtctatgccggcggggaagtaaaaaataagttcatcataagcgaaggcagggtgtacatcctgccttcgtattttattgttagattgaagattttgctatacgctggggctgattatgtgatatactaacaaaaacaatagcgattgcacatgtggaggagatagcctggtttcgcgtcatcggcaagggtgactctacaccctaaaatcgagagagtgcgcaaaaagcgcggaatcatcgcttgcgaatacactcgataaggtagaaattgtgcatatggattccatgcacacagctcattttagtagcttttgccgacgcacaccgcacgcgggtatgggctgagagggtgatcgacagcaacaagtgagcggacgcaactgacgcacaccgcacgcgggtatgggctgagaggtcagcggatactgcgccgtgcctgtgccaatggtgacgcacaccgcatgcgacaacacctctgcaaaaaagtttccatgaacccttgacaacgagcattctatcgtctataatatcatctgtttgaagcagaagcgtgcccgcttctcgccctgtgacttgcgttgctgggctgatggcaaaaaggttttcgtgtgaaaatctgactacgtcatgacacagcgggtgaggcttctccccgctgttttttcatggaaagcggcggtcagacaattttgaggaggtgc

SEQ ID NO: 60 - DNA, 1712 bp, synthetic construct
  source 1..1712: mol_type = other DNA
cctttatatcccactacgttcatataaaactgtgatcgacagcaacaagtgagcggacgcaactaatcctttatatcccactacgttcatataaaacttgttcttttgttgatagtagtttaattttaactgttattgtttgagacattgttctacacctgtatctctaatcatttttgctctttttatacttctatactcttctaaagttgcttctcttacaatagaccaagaaccaagccacatcatttcttttatacacccgttaggtattttaatttgtgatgtatcacactcattcctgccacatagaactaatatggctctttcgtagtcggctctatattctttatcaaatttatggtcttttacaaactgttcaaaatcacagttactacatttcacttgcatatcttttacccccttgttttttgctgttcaacataccgtttaatcgtttctcttgatacgtttcctgcggtagaaacgaaataggaacgtgtccataggcttggcaagtgtcgaagatgaggaaattcctctctcagctttttcgaagtcactcctttgatttttgccatgatatcggaaggactaaatgttggtagtgcatttaggaacatatgtgtatggtctttatcacattctaaagcaataatgacaatttccaattcttcgcatatttcctttactaactgtttaaaacgttcctctacatcggtacgaagaaatattttccttctgtatcgagggcaaaaaacgaagtgataattgattaaagatacggttgtatgagttcttctatattcgttcatactcatatcgtatcagtttaatctacatacagcaacgaaaatacaaaaatatttggaacatttgacgtggcataaagccacgcctgttccaacctcactctcatcccacccctaaaggagtgggctttctcgctcagaaaatctgtaaagaaaggtatctatcatatccaacatgtgaattcgtatcacagtcgcctcaaaaattggatgaatggatttaatggtgtggctacacgatacttggataactatttattttagttccgtttcttagagataaataaggaaattggagaaaaaatgaccccaaaagcaatgcttatagcatcatgtcaaaagccaaattttacgaaagtaggttcttttcggcacgttagtttacatctaacttaaatttctgacgactacctccttctgaaataacaccctttcgtttacaatattcaccacttagtcatacgactatcttaaaccgatgcaatcataccatttttaggataatcccactactgtcatctataaagcaacaattttttagaaaaaagcgaaagaaaaagatcctttatatcccactacgttcatataaaactgtgatcgacagcaacaagtgagcggacgcaactaatcctttatatcccactacgttcatataaaactccctaaaaacaaaacggacgaaaaccttcatctatcaaggatttcatcgttcaaagaactcagcaaaagtcggctttttgcagtaaaccaggaattctatttttcacataggagaaaaaacgcctcaaatccttgctatataaggcctcatgtccagtatacccaaaagtaggtttactgcaaatcatgaacgtattccgccacgaacaccgaatatgaagaatgatatctaagtaactt

SEQ ID NO: 61 - DNA, 629 bp, synthetic construct
  source 1..629: mol_type = other DNA
actaacgtatgtaatgattgattactaacgtatgtgataagcaactacatgcgttagcaataatagcccttataagtatattaaattataaccaaaatcagtaaaaaagacacgattatcaacacccatgcgtacatcatcgcagatgactttatagttggatataccatacaaaacaataataaaaccaacgtgatcgacagcaacaagtgagcggacgcaactaaatataccattcaaaacaatgataaaaccaacgtgatcgacagcaacaagtgagcggacgcaactaaatataccattcaaaacaatgataaaaccaacatttagtttctaagtttattaatttcaatgttttgacgtacttcccgagtatagtttcctatctcaggttaaggacttccagcagccccaattagaaaatttcttttgtgtaataataggcatactctttttaattttaccaccgcaaatattgtaattataattgtaagtctcaaatccaactcaaataatttcctataaaatctatcggcaagtttatataatagaatatcatggcaaagatacattttttgccgatatcggcaatatttcaatcaaataaagtcaggctattatccacctgt

SEQ ID NO: 62 - DNA, 813 bp, synthetic construct
  source 1..813: mol_type = other DNA
gaagcacttcacagaagtgcatggagcagaaggtgatcgacagcaacaagtgagcggacgcaactagaagcacttcacagaagtgcatggagcagaagcgcactccgtctctgccctgtcaaggcagctgttttgcaagttcgattatacctttggggtaaatggttgtcaatggcgggcccgcgacagaaaataggaagcctttctctgcacattcaacaaacaacatttacagaatgccccaattatgttatactaatgttgccttgcaataatgtgaacgtgaaatggagggatgtctgtggcagatatcaaatctcaaagtggtgggaggtctgtccccaccatggggtgcgaaccttgtgtgctcatcattgccgtgagcgttcgcacgtccaaacgaccatatcatcgttgccctgcgaccattcagcggcaatcaagacgcaggcatgatatgtaaccatgcatttctgtgaactgcttccaaaacgcactgcttcattataatcctccctgtgcagttctgccgaagcacttcacagaagtgcatggagcagaaggtgatcgacagcaacaagtgagcggacgcaactagaagcacttcacagaagtgcatggagcagaagaagtcgtttatagcggtttgtttacagggagttagaagcacatttcaatttttcagtaaaactcctccagctttgcagctgggggagttttttactcccctcttgacaattatcttctacgtctgtagaatataatcaaactacaaccgtagaagatattcacagaagggaggataacgctatg

SEQ ID NO: 63 - DNA, 807 bp, synthetic construct
  source 1..807: mol_type = other DNA
cttctgctccacgcactcgtgcggaatgcttcgtgatcgacagcaacaagtgagcggacgcaactaatcttctgctccacgcactcgtgcggaatgcttcggggtccgtaagcgagactgataccatgagaaaaacgagcgccgtggggagccacggcgctcgttcttttttgttgggggttgagaaaggaccgccggtatcccggcggtcctgcttcgtttacagaatggagcgaggatatggcacctctctcgtgcggaatgcttccttgcggctgccaggcagatgcgcatcgtcgtaggtcttctgctccacgcactcgtgcggaatgcttcgtgatcgacagcaacaagtgagcggacgcaactaatcttctgctccacgcactcgtgcggaatgcttcggcaagatcctacgatctcatggctgcgagaggacgacgcggaagcagtctgcacgaatgcgtggtcccatatcatacccgcgcgcggatcgcccactcgaaatggcgcgcaagatagcgatgatatgtctgttcggaggtgcgaacacccgcggcgaccggcgggcgatcaaggttcgcactcctcggtggggacagacctcccaccgatgttctcatttccttgtttcgttctgttcgtttcgttcgatgtagctcctcacctcccatgctacatcatccgacgcttggtccttttcggtcccatcataccacgctgcgccagagctgtaaacaccgagaccgtcctaagatgcagaaaggaccgccgggatgtcggcggtccttctctttatctcgtcct

SEQ ID NO: 64 - DNA, 853 bp, synthetic construct
  source 1..853: mol_type = other DNA
ctttcaattcacgacctcccgaggaggtcgacgtgatcgacagcaacaagtgagcggacgcaactactttcaattcacgacctcccgaggaggtcgacttttttcgattgtcaatttcttttggcaaatgactatatttcatttttaatcagtgcaattttttccaatttctcggattcagtgtatcgcggaattttaatttcttattatattttttctcgtaatcctttttgtttaatctgtatacacaataccacagaagtagcacgattattagccctgacatagtatttaccccttttcaactcacaacttcttaataaaaatcacgctgctgcaaaccttattgcagaatttctactcacacgtcccttacgggacgtgacatcttccgatttaatagagacattgtggaatgtaatttctactcacacgtccctcgcgggacgtgacgtcggatgatttgaatatagaaacaaagagtaatccatttcaattccagaccttccgagaaggtcgacaacatgccgctcatatccgtcacctgactggtatcctttcaattcacgacctcccgaggaggtcgacgtgatcgacagcaacaagtgagcggacgcaactaatctttcaattcacgacctcccgaggaggtcgactgcaaaattccacagttttcatctctaaaaccttgaaattttttaatacctttactaatttctcttactccttcttgctttaataccactcattttcccttttcctaactaaaacctctccattttctggtgcgaatgccgaagacttttctgtgtgcttaggattcgcgctccacttgaaacatgttctgacacgg

SEQ ID NO: 65 - DNA, 697 bp, synthetic construct
  source 1..697: mol_type = other DNA
gtccggtccgtgcgcgtggggagcgaccgtgatcgacagcaacaagtgagcggacgcaactgtccggtccgtacgcgtggggagcgacgaacggatccacagcgggcccttgatgacccgacagaaaggcacctttcgttgagaaacaggctctcccgcccccctgcggctcaaggcccgagaaccggccttcgctactggctcgcccgccgccgccgggccatggccgcacatgcactgcgcggcgcctgctacggcatcggcaccggcgcagtcggcctcgtattctggtggatcgagcagaccctgtaaacgggctcccgcacccaagggcagggcgggcggcgcgggtgatctggtggtgaagaagcaggtcagcggccgaacggggaccgttgtcagtggtggcctctacagtcgtcaacgactcttggcgcgcgggtggttgaaggaggtggctgatggcggagacggcggtgctgcgtgcgaccagcaaacggcaaagcggccctgaaaccgcaggtggcgaagtgtccggtccgtgcgcgtggggagcgaccgtgatcgacagcaacaagtgagcggacgcaactgtccggtccgtacgcgtggggagcgacgagttgctgttgtgcctgcccgcatgccgtcttggtctaggcgatctcccagcggttgctgtcgtgggtctgttcgt

SEQ ID NO: 66 - DNA, 1242 bp, synthetic construct
  source 1..1242: mol_type = other DNA
ggtcggcatttacacgaaaaccaatgcagttacaacagtgatcgacagcaacaagtgagcggacgggtcggcatttacacgaaaaccaatgcagttacaacacgaacggagcgttcgcgtcggttttgattccgctccggttttcgctccgcgtggaatcacgttccgttctcggttccgtattattcggaaattccgccctatctgacaggggcggaatttttttgcgcgcgtgcttgccggctgcgcgaatcatgtcggttaggttgagcgaatcatgccggttattgtgtaaggtttttgcggcaaacgtattgtttgccgcaaaagagaaagtccctaatgtccttaaagtcattaaggactttaatgtcgttaatattgtcgtgcggcgaatatttgttcaccgcttttaaaacctttaaagaccctaatgtccttaaagactttaaagtccctaatgccgttaaggactttaatccccattctccctccccgcctaattctccgcttccctgtcgcggcggtcgaagacatcgacggtgaggtcggcatttacacgaaaaccaatgcagttacaacagtgatcgacagcaacaagtgagcggacggttggatattcacttgaaaatcaatgtggttacaacatgaaaactgtaacatgatgatatccaatttatattataaaaaatcaagtgaacttttcgagtgcagggacatccgtaaaatattcattatgcggattatggtgtcctcacctcaaaccaaggcgctccaacgcgcccatcccgaaagggattatatcgttacatatatttatcgtataaaacaataagtatcattagttcaagtgcaggattccgaaaaattcggattttattttaaagaccgacacaactgttgcaaagatagtatatttagtgggttgttgcggttagttttcttctctgtcgcggcggtcgaaggcatcgacgatatgcttgacaagttcgtggcggacgatgtcgtgcttgtcgaactcgacgaagccgatgccctcgatgccgcgcaccgtctgcatcgcgcgcaccagtccgctgtcgctgcgccgcggcaggtctacctgcgttacgtcgcccgtaacgatgaacttcgcgttgcgccccatacgcgtcaggaacatctttatctgcgacatcgtcgtgttctgcgcctcgtcgagaatcacgaacgcgttgtcgagcgtccgtccgcgcatgtagg

SEQ ID NO: 67 - DNA, 847 bp, synthetic construct
  source 1..847: mol_type = other DNA
ttaaatataacctatgttaatcattaacgtgatcgacagcaacaagtgagcggacgcaactaatttaaatataacctatgttaatcattaacgtactcattttaaatccccctcattttaatcttacattaaaaattttacctctttaactgttttctgtacacaaattcgacaaatttagaattaaacatttattattagacaattatttttaataaaaaatgagcctagaagtaactaaactcctaggctcatttcgtgcaatattcttattatatttataatttattttaacataattctattatttattaaactacattaaccattaaatttacattcatattcaacataatctatgttaatcattaacaaaggaggttgcttatgtttaataacaatatttcatttaaatataacctatgttaatcattaacgtgatcgacagcaacaagtgagcggacgcaactaatttaaatataacctatgttaatcattaaccttagtaactcagccatttcctctaataattattaatttttctaattggttatatcatagtacccaccatgcttatagcattttttatactagctttttaccagcaaatttcaactggagcggttgtaagagtgttaacatgcttcctttcaagtaatttcaatgtttttaagcgtgttacttctctacttaggatggtaaatcaccctttattaaaatcatttactccctcatttcaaagttttatttttaaagttttataaataaaaaaagaagacctagagattccccctaggtctattatgtgcaacatttacttatattattataaaaattatattttaaa

SEQ ID NO: 68 - DNA, 1302 bp, synthetic construct
  source 1..1302: mol_type = other DNA
gacgaacctgggcatcaccaccggcgacctagacggtgatggccatccggagctgatcggggcgggctataccgactcccgcgcgcagggatgaaccctgtgatcgacagcaacaagtgagcggacgcaacccgactcccgcgcgcgcagggatgacccaaaagcacgcgggccgtaaagatcagcgcaaagccgactcccgcgcgcgcagggatgacccgtgatcgacagcaacaagtgagcggacgcaactccgactcccgcgcgcgcagggatgacccgctgcgcaaggtgtgcacaccagcggtcggcgcgcggggctctccctgcaaagcacggattccggggccgatcgctccaatgccgcaaccgtctacgtgcaggcggcggcaccacccgcgatcgtatctcctccggcgtcacttcgccccgttgaatgtatgcgcattgatttcatggtgccagggcgcgactttatcgcgttcctcacgccagtagtagaggatgcgcttgccgattcctccctttccctgcttgaaaaactcaaatcccttttctcgcaccagacgtagcgcccagttgtagatgaagcgcgccgcgccgaaatgctgatgcaggaagcgcctttttctctcagaagcaatttcgagctcaagacggtaggcgcgcagcatacttgctccggtgcgtatatgcttgtgacaggaatatatcttgtaattggctacatgtcaacgacatatgtccggaggctcatcttcagaaagtgtgtgttggagtgtatcatagaagacccaggacgcattcgagtactcggagtagaaggccatggagtttctcatcctggatttgatggacatggaagaaagccggcggtggattgcgcagcacttccaccccgaaggccttcgctgtcctcgctgtcaggccttggtcaccgaggcccgtctgtttcgccataccaagcggagtcaactgccagtctaccggtgcaaacggtgtgggcgaacctacaacctgtacaccggcacggtgttcgaatttgacccctcagcaggtggtgttgctgctccgggggatggccaaaggggaaagcacccaggtgctggcggccgaactggggttgagttatggcacggtgttgagcttacgccatgcgcttcaagcccgagcggcggggctgcaaccggagaggccgctgccggatgcggaagtggaggccgacgagatgttccagaatgcgggggaaaaaggcgcgccgcatcggcatcccgacgacccgccccggcggcggggaacccg

SEQ ID NO: 69 - DNA, 2075 bp, synthetic construct
  source 1..2075: mol_type = other DNA
atttaaataacatcatagtgctattaaaccgtgatcgacagcaacaagtgagcggacgcaactaaatttaaataacatcatagtgctattaaacccttttaactagttagtagtttttagatagtagtttttagttatgattgaaagattaaattagtaacaagttacaagtaataagtgacaagtttaggttgaaactcctttattagaaactcctttaggagtttctaataatatattttcaaaaattcagcataagctgaatttttcagactgttgacaaagtgtcagcagtctgataattattatttaattaaattaatattttaaattcatataatccctatatctcttattatatcaaggttaaactgataaattttagtttaatactacttaaataatgggagttttatttcctataacttatactattttaaataaaactcttattatttattgctactacgtcttaagttaatagtctcattaataataaaattatatccattattaaacatttaaatcaaaaaaatagaaaacattaagtgattcctaagaatcgtttaatgttttctatttttacatttattcaataattattataattctcatcctatatataatatttttataatttacagtatcacaatttcattaatttaaataacatcatagtgctattaaaccgtgatcgacagcaacaagtgagcggacgcaactaaattaacattccattatggcgctattaaaccccgttaactttaaagccactatatatctagtttgatatagtagtttctgtctacctcttattttataataaattttatcaatactaattaccaactttaattataaaatagctaccctgtacttatattacttattttgtctaccacctgtgtttttaccctatctatgatagacaataaactaatataattattcaattttggaacgcctaacggtcacacattgttaagattaacccttaccgagtgattatggtatatagttggtcaaaaccttatatatttaatccatctcctcagccttcggcactttaagttaccgtaactgctatatatttatatataacatcaatacaattatattacattattttgaatttgtaaataaagattagttttatcaatgtattaatttaaccttccttactgttatcatttctatatatcctcataaattattttttattacaattataccatttttacataattatatctataattaatagtttctatacattattttttactacattataattttattgctaaaacgtattaatataaatgtatatctataaagaaaaaaggctataaatttatagccaaatgaataaaaaataaatttaagtaaataatataaatgttagtttaagaaagcttcttagatatttgtttaactggatgcttaccagtagatctaagagcttttttgctttttttataatatgaattgtttcttttattttttttcctttttcacattgtattcaaatttatatatgtaataatgaattacaattgtcagtattactacaataaggaagtatatgctccatttcaaaaaagcaaaaaaagtttatctcctaaattcatctttatctcaccttctttcttaagttaatttagagtttttgctcatttaattttccccctgaaatttatagtgtcaattctacaacgcccttccccagctacgctgtgttgttttttgacactgcctaaaaatcacatggagatatacttgtcaaaaattaaagcatctttaaaggagttggttttattcagtttacacaaaattttttacagggcccttcaataaaagagatggccctaagccatcttttttcacatttattacaattaaaacatttaaaacattcaaaaatccgatattcttgaaaatcttccattccaccttaatgcacatgtacccctttcaccatgcctattcttaataattacagcattaatacattcatgattttcatcagcatttttagattcatactttaacttgccaagcctaaacagcttgtc

SEQ ID NO: 70 - DNA, 1269 bp, synthetic construct
  source 1..1269: mol_type = other DNA
gatgcattttatatatataagtggattgaaatcgtgatcgacagcaacaagtgagcggacgcaactgatgcattctacatatataagtggattgaaataccaaacagaaaaaatacaagccaagaatattaaaagaattatttgaataaaaggagaaatgtaaaatgaaaacatttttatttatagcaggtttttgcttagaagttgcatgttttaccactattataaatctgtacgactggaaagcttttgcattatcaataggagctgctcttggtgcatctatagttggtataatgaggaataaattggatagataatttaaaaggagagaaaatgacaatgttaatatatggttgcaggttcaacgccgccaagtgcgaatataaagtacacataaattacatggcaattcgcactaaagtagataaaagaaatttgatagtagtatatatactatgattactatcactatatatacgaaacaaaatattgcttttataaccataacattatgtaaattatacaaaatatgatagtcacatttatgtatttttgctgatgtaatttacatatatgtgtggattgaaatcaagggggtgctaaaatggaatatctcttttttagaggtaatttatatatatgtgcggattgaaatcagaagttccaccagtattttttctggctgcgaggtaatttgcatatatgtgaggattgaaataagttttagtacactaaagcgtttaaaacaatagagatgtaatttacatacatgcgtgtattgaaattacctgtctagggcggtagcctataaattatagatagaacttacataggtaagattattatatctcagacaagtaaaataacatgactaatattataaatattataaatattatatataaaatataggtaggaggttcaaccccaccttggtgcgattagacagtgaacatatatttcttaatagattcgcaccagaagtagataaaagaaatcagttagtacgatagttaatcatagcaatatgttaattattcgaaaacagataatgcttttataaccacaaatatgtataaaatgcacaatgataatagataagtcttatatatatttgctgatgcattttatatatataagtggattgaaatcgtgatcgacagcaacaagtgagcggacgcaactgatgcattctacatatataagtggattgaaatatttcacaatatacacaaaaataaaaggagtataataaaaatgacaata

SEQ ID NO: 71 - DNA, 940 bp, synthetic construct
  source 1..940: mol_type = other DNA
aaaaatcgtgaaagataattagaaaagaaattttctaattggggctgctggaagtccttaacctgagataggaaactatactcgggaagtacgtcaaaacattgaaattaataaacttagaaactaacggttggttttattatagttttgaatggtatatccaacagtgatcgacagcaacaagtgagcggacgcgttggttttattattgttttgaatggtatatccaacagtgatcgacagcaacaagtgagcggacgcgttggttttattattgttttgaatggtatatccaacagtgatcgacagcaacaagtgagcggacgcaattggttttattattgcttttgaatagtatatccaactataaagtcgtctgcgatgatgtgcgcatgggtgttgataatcgtgtcttttttttactgattttagttataagttaatatacttataagggatattattgctaacgcatgtagctgtttatcacatacgttagtaatcaatcattgcatacgttagtaacaagaaacgactaacgtatgtaataatctgcaagaaaactttgccatttcaaataaaattgtaattttgtcattacagtccccactaataaaaaaggaggtcagtaatgctgttcatggtgaaatggctggaacgtgtagcaaaataaatttctcgaaatagaatttacttgtggaatccctcatgcggttgcatgggggattttttatgggcgattttgagaatttttgaaattctgaaaattatttgagttggatttgagacttacaattataattacaatatttgcggttgtaaaattaaaaagagtatgcctattattacacgtaagatagaattgaaaatcgtaaaagatggattgacagatgaagaatatgaccaacaatggaaatatctttaccagataaacaacacc

SEQ ID NO: 72 - DNA, 1187 bp, synthetic construct
  source 1..1187: mol_type = other DNA
gttgcaattcgtatgcgcaggtaagtttcgaggtgatcgacagcaacaagtgagcggacgcaactaagttgcaattcgtatgcgcaggtaagtttcgagtactgatttttaatcaaagtgtagacagtgtagacaaagaatctgcgccaagatatataaaccggtttttaacataaacctgttttcaacagctacgagcttttgcttgtttttgtacactttgagtttaaaaatagtataaaagctgattctatgtgcataatagctatagtaagatactgaaattcaacttttaactgtataaaatgacaaaaagcaaaatttctcgaaaatattttaaaaaagctattgacacatagcccctttaatgctataatgattaagtcgcacagagagaataacaaaaaagctgctgaagctttgcggcaattgtaaatggcggcatggctcagttggctagagcaaccggttcatacccggtaggtcgtaagttcaagtcttactgccgccaccataataaggcccgttggtcaagaggttaagacgacgccctttcacggcgtaatcatgagttcaattctcgtacgggtcaccaaaatccgaacactttcagtgttcggatttttttgtttaattattaaattataatttgattcaacatcgttcattaaaatattattggtaaaaaaacacaaaagtaaaataggtgtttgtttatattgtcaattgaatctataaaaataaaatgataaaataattatattatttttttacgcaaaatcattgtggcaaaaagccaaaagttttgattgtctacttataaggcgaggaaaatgatattggtgcgaatatagagtacacataatttattagaatattcgcactcccaaaaggggcggctcggcgtcccaaaatcgagaaagtatatgtaaatctgaatttattcagtagtagatacactcgataaggtataaacaatacacattttaatccgtgtattgaacttatttagctattttgcagttgcaattcgtatgcgcaggtaagtttcgaggtgatcgacagcaacaagtgagcggacgcaactaagttgcaattcgtatgcgcaggtaagtttcgagttttaataacagatatttaaactcctgtacaacccaaaaggtgttcgggagtttttaattatattc

SEQ ID NO: 73 - DNA, 1258 bp, synthetic construct
  source 1..1258: mol_type = other DNA
atttgattagaaccatattggaatgtaaatgtgatcgacagcaacaagtgagcggacgcaactaatatttgattagaaccatattggaatgtaaatataaagaaaataatggctgttgcatattttgcagcagctttttttcgtctaagttaaaataatatccctcttgctctccagacttcgacgcctcgtccattaaactaacacatttaaatgttacgaggcgtctatagattgtcgaattgagaggggtatttattttaaaaataaccaaagaataatctctgcaaaatattgcatacagccattatttaataagtagataattattttatatagtagaaaaaattctgtttaaaatatataatgaatataaggaaataaaaatctgcgaaacatttaatattaaaaattgtgtttgatatataaaattataatgtgtatataaatttgtggggagtaaattataattatctacttattaaataatggctgtatgcaatattttgcagagattattctttggttatttttaaaataaatacccctctcaattcgacaatctatagacgcctcgtaacatttaaatgtgttagtttaatggacgaggcgtcgaagtctggagagcaagagggatattattttaacttagacgaaaaaaagctgctgcaatatttatataatttttaaataataatggttctataggcgatttagcgtctaaaggttgagggataagacaaaatggttaaggtttcgaccaactaactacttatccactcgataaacggtaaaaactcatactaatattctttatagataacgtggtatgacattccaagaattatataaattgtcgaccttagataatgtaaaatacctaggagatagacaaaatgagatattgcaatagttggatctgttttttatcaagaaggactattttttactttagaaaatatatgtttatttgtaggtagacaaatagtatatctgtatatgttgcaattgctaggtttaatatataacgtatttgattagaaccatattggaatgtaaatgtgatcgacagcaacaagtgagcggacgcaactaatatttgattagaaccatattggaatgtaaattatgtattgcatattgttgaccaaggtcctattgaatctgactagaactattttatgacaattatgcaaattaatattttttagccaagaaaaccaacatacgaaagttttcttggctattattttaaata

SEQ ID NO: 74 - DNA, 1704 bp, synthetic construct
  source 1..1704: mol_type = other DNA
tttgagaatgatgtaaaaacgtatggtactcagtgatcgacagcaacaagtgagcggacgcaactatttgagaatgatgtaaaaacgtatggtactcagtttgaaaaataatagttgacgttggttattcaaaggggtatattataattagttttgtaccatacaaaattacatcataagttcaaataacgatttatcgtaaacgccgcgtgtgcggctcacagtgtgtgaaaaagtaactgctattcggaatcagagtggcagtttctttttacataaatataaacagagatgaagaatgtgggaaaataaaatttgctattggtaaaagatataaaggaggaaactttaagtaactgaataagttgtcagatgtgataatatgtgtttaaatatactcatggaggtatactatgaatacatcaaatatcacaaattacaagccaaaagattttgctgaattgctaggtgtttctgtcaaaacgttacagcgttgggatagagaaggaactctaaaagcaaatcgtactccaactgataggcgttagtacacttacgaccaatatcttcaattcaaaggcataaatacagaagatgatacgcgtcaagttgtcatttatgccagagtctctacaagaaatcaaaaagatgatttacaaaaacaagtcacatttctacgacagttttgtaatgctaaaggtattatcgtagaccaatgtattgaagattatgggagcggccttaattacaatcgcaagaaatggaacgaattattagatgaagtaatggaacagaaaatcaaaaccattatcgtaactcataaggatagatttatccgatttggctatgattggtttgcaaaattctgtatgaagttcaatacaaccatagtggtagtaaacaatgaagaactatcgcctcaagaagaactcgtgcaggatattgtttcaatactccatgtattctcttgtaggttatatggacttcgtaaatataaaaaacaaatagaaagggtcaaacgcaaacgtaagtatgtaccgaaggcttattcgggaattaacgactgtggagtgtacaagaacctgcaagtagatatgatttcggtcaatcaaaagcatacacgatgaagcagtaagtagagttcgtgagaacctatattatctcgatgtgcgtatatttacacacattttgagtggcagaatgtaaaacgtttgagtaccatgcccggtgcggatgaggcactgcatttttgaactttgaggtttgagaatgatgtaaaaacgtatggtactcagtgatcgacagcaacaagtgagcggacgcaactatttgagaatgatgtaaaaacgtatggtactcaaacatctgtatgtcagatctggcttgtggctcagtttgagaatgatgaaaaacgtatgctaaactgaagcgtaccaaaaagtgttatccgcgtttgagaatgatgtataatttgatttcttaaaaaacttctatgtcgccatccaataggtggcgaatttcttatactcaatatatcgtatatcgcatttagcgtttttaattaatgtaattaaattggagaatgtggttttgagaatgatgtaatattgtaaaaatatttgttgtgggacattatgagaatgtctgcgcaatattgagtttatagtcgatattatttgagttcaataaaagggagtttttatg

SEQ ID NO: 75 - RNA, 230 nt, synthetic construct
  source 1..230: mol_type = other RNA
gccttgcaataatgtgaacgtgaaatggagggatgtctgtggcagatatcaaatctcaaagtggtgggaggtctgtccccaccatggggtgcgaaccttgtgtgctcatcattgccgtgagcgttcgcacgtccaaacgaccatatcatcgttgccctgcgaccattcagcggcaatcaagacgcaggcatgatatgtaaccatgcattggaaagtgcatggagcagaag

SEQ ID NO: 76 - RNA, 168 nt, synthetic construct
  source 1..168: mol_type = other RNA
ggtgggaggtctgtccccaccatggggtgcgaaccttgtgtgctcatcattgccgtgagcgttcgcacgtccaaacgaccatatcatcgttgccctgcgaccattcagcggcaatcaagacgcaggcatgatatgtaaccatgcattggaaagtgcatggagcagaag

SEQ ID NO: 77 - RNA, 235 nt, synthetic construct
  source 1..235: mol_type = other RNA
ggtgaacattcgctacgcaactgtggttggcggtaatagtcaatcagcctaagaacctatatggtctgtcttaggaggggtgatggcacaccctcatcttgaaggctgttcaaaacagaaatggactgcgaacgtttagtcattcaagaatcccatccgttacaccataaggtgtaggacttgcggctttagccgtgggagtgtcaaaaaacacagtaggagggacttacgttag

SEQ ID NO: 78 - RNA, 102 nt, synthetic construct
  source 1..102: mol_type = other RNA
ggttctgcatggtcagaatcggaatgggtcaaagagcagctacaagcccatgacttcagtcgtgggtagttgacaaaacacagtaggagggacttacgttag

SEQ ID NO: 79 - DNA, 24 bp, synthetic construct
  source 1..24: mol_type = other DNA
gtgatcgacagcaacaagtgagcg

SEQ ID NO: 80 - protein, 575 aa, synthetic construct
MSVSFSLNAKKIRLENYAMKMRLYPSPTQAEQMDKMFLALRLAYNMTFHEVFQQNPAVCGDPDEDGNVWPSYKKMANKTWRKALIDQNPAIAEAPAAAITTNNGLFLSNGQKAWKTGMHNLPANKADRKDFRFYSLRKPRRSFAVQIRPRCIIPSDTNQKVARIKLPKIDGAIKARGFNRKIWFGPDGKHTYEEALAAHELSNNLTVRVSKDTCGDYFICITFSQGKVKGDKPTWEFYQEVRVSPIPEPIGLDVGIKDIAILNTGTKYENKQFKRDRAATLKKMSRQLSRRWGPANSAFRDYNKNIRAENRALERAQQDPGSSGVGPEAPVLKSVAQPSRRYLTIQKNRAKLERKIARRRDTYYHQVTREVAGKSSLLAVETLRVKNMLQNHRLAFALSDAAMSDFISKLKYKARRIQVPLVAIGTFQPSSQTCSVCGSINPAVKNLSIRVWTCPNCGTRHNRDINAAKNILAIAQNMLEKKVPFADEALPDEKPPAAPVKKAARKPRDAVFPDHPDLVIRFSKELTQLNDPRYVIVNKATNQIVDNAQGAGYRSAAKAKNCYKAKLAWSSKTNK

SEQ ID NO: 81 - protein, 575 aa, synthetic construct
MSVSFSLNAKKIRLENYAMKMRLYPSPTQAEQMDKMFLALRLAYNMTFHEVFQQNPAVCGDPDEDGNVWPSYKKMANKTWRKALIDQNPAIAEAPAAAITTNNGLFLSNGQKAWKTGMHNLPANKADRKDFRFYSLRKPRRSFAVQIRPRCIIPSDTNQKVARIKLPKIDGAIKARGFNRKIWFGPDGKHTYEEALAAHELSNNLTVRVSKDTCGDYFICITFSQGKVKGDKPTWEFYQEVRVSPIPEPIGLDVGIKDIAILNTGTKYENKQFKRDRAATLKKISRQLSRRWGPANSAFRDYNKNIRAENRALERAQQDPGSSGVGPEAPVLKSVAQPSRRYLTIQKNRAKLERKIARRRDTYYHQVTREVAGKSSLLAVETLRVKNMLQNHRLAFALSDAAMSDFISKLKYKARRIQVPLVSIGTFQPSSQTCSVCGSINPAVKNLSIRVWTCPNCGTRHNRDINAAKNILAIAQNMLEKKVPFADEALPDEKPPAAPVKKAARKPRDAVFPDHPDLVIRFSKELTQLNDPRYVIVNKATNQIVDNAQGAGYRSAAKAKNCYKAKLAWSSKTNK

SEQ ID NO: 82 - protein, 575 aa, synthetic construct
MSVSFSLNAKKIRLENYAMKMRLYPSPTQAEQMDKMFLALRLAYNMTFHEVFQQNPAVCGDPDEDGNVWPSYKKMANKTWRKALIDQNPAIAEAPAAAITTNNGLFLSNGQKAWKTGMHNLPANKADRKDFRFYSLRKPRRSFAVQIRPRCIIPSDTNQKVARIKLPKIDGAIKARGFNRKIWFGPDGKHTYEEALAAHELSNNLTVRVSKDTCGDYFICITFSQGKVKGDKPTWEFYQEVRVSPIPEPIGLDVGIKDIAILNTGTKYENKQFKRDRAATLKKMSRQLSRRWGPANSAFRDYNKNIRAENRALERAQQDPGSSGVGPEAPVLKSVAQPSRRYLTIQKNRAKLERKIARRRDTYYHQVTREVAGKSSLLAVETLRVKNMLQNHRLAFALSDAAMSDFISKLKYKARRFQVPLVAIGTFQPSSQTCSVCGSINPAVKNLSIRVWTCPNCGTRHNRDINAAKNILAIAQNMLEKKVPFADEALPDEKPPAAPVKKAARKPRDRVFPDHPDLVIRFSKELTQLNDPRYVIVNKATNQIVDNAQGAGYRSAAKAKNCYKAKLAWSSKTNK

SEQ ID NO: 83 - protein, 575 aa, synthetic construct
MSVSFSLNAKKIRLENYAMKMRLYPSPTQAEQMDKMFLALRLAYNMTFHEVFQQNPAVCGDPDEDGNVWPSYKKMANKTWRKALIDQNPAIAEAPAAAITTNNGLFLSNGQKAWKTGMHNLPANKADRKDFRFYSLRKPRRSFAVQIRPRCIIPSDTNQKVARIKLPKIDGAIKARGFNRKIWFGPDGKHTYEEALAAHELSNNLTVRVSKDTCGDYFICITFSQGKVKGDKPTWEFYQEVRVSGIPEPIGLDVGIKDIAILNTGTKYENKQFKRDRAATLKKMSRQLSRRWGPANSAFRDYNKNIRAENRALERAQQDPGSSGVGPEAPVLKSVAQPSRRYLTIQKNRAKLERKIARRRDTYYHQVTREVAGKSSLLAVETLRVKNMLQNHRLAFALSDAAMSDFISKLKYKARRIQVPLVAIGRFQPSSQTCSVCGSINPAVKNLSIRVWTCPNCGTRHNRDINAAKNILAIAQNMLEKKVPFADEALPDEKPPAAPVKKAARKPRDAVFPDHPDLVIRFSKELTQLNDPRYVIVNKATNQIVDNAQGAGYRSAAKAKNCYKAKLAWSSKTNK

SEQ ID NO: 84 - protein, 575 aa, synthetic construct
MSVSFSLNAKKIRLENYAMKMRLYPSPTQAEQMDKMFLALRLAYNMTFHEVFQQNPAVCGDPDEDGNVWPSYKKMANKTWRKALIDQNPAIAEAPAAAITTNNGLFLSNGQKAWKTGMHNLPANKADRKDFRFYSLRKPRRSFAVQIRPRCIIPSDTNQKVARIKLPKIDGAIKARGFNRKIWFGPDGKHTYEEALAAHELSNNLTVRVSKDTCGDYFICITFSQGKVKGDKPTWEFYQEVRVSPIPEPIGLDVGIKDIAILNTGTKYENKQFKRDRAATLKKMSRQLSRRWGPANSAFRDYNKNIRAENRALERAQQDPGSSGVGPEAPVLKSVAQPSRRYLTIQKNRAKLERKIARRRDTYYHQVTREVAGKSSLLAVETLRVKNMLQNHRLAFALSDAAMSDFISKLKYKARRFQVPLVAIGTFQPSSQTCSVCGSINPAVKNLSIRVWTCPNCGTRHNRDINAAKNILAIAQNMLEKKVPFADEALPDEKPPAAPVKKAARKPRDAVFPDHPDLVIRFSKELTQLNDPRYVIVNKATNQIVDNAQGAGYRSAAKAKNCYKAKLAWSSKTNK

SEQ ID NO: 85 - protein, 575 aa, synthetic construct
MSVSFSLNAKKIRLENYAMKMRLYPSPTQAEQMDKMFLALRLAYNMTFHEVFQQNPAVCGDPDEDGNVWPSYKKMANKTWRKALIDQNPAIAEAPAAAITTNNGLFLSNGQKAWKTGMHNLPANKADRKDFRFYSLRKPRRSFAVQIRPRCIIPSDTNQKVARIKLPKIDGAIKARGFNRKIWFGPDGKHTYEEALAAHELSNNLTVRVSKDTCGDYFICITFSQGKVKGDKPTWEFYQEVRVSPIPEPIGLDVGIKDIAILNTGTKYENKQFKRDRAATLKKMSRQLSRRWGPANSAFRDYNKNIRAENRALERAQQDPGSSGVGPEAPVLKSVAQPSRRYLTIQKNRAKLERKIARRRDTYYHQVTREVAGKSSLLAVETLRVKNMLQNHRLAFALSDAAMSDFISKLKYKARRIQVPLVAIGTFQPSSQTCSVCGSINPAVKNLSIRVWTCPNCGTRHNRDINAAKNVLAIAQNMLEKKVPFADEALPDEKPPAAPVKKAARKPRDAVFPDHPDLVIRFSKELTQLNDPRYVIVNKATNQIVDNAQGAGYRSAAKAKNCYKAKLAWSSKTNK

SEQ ID NO: 86 - protein, 575 aa, synthetic construct
MSVSFSLNAKKIRLENYAMKMRLYPSPTQAEQMDKMFLALRLAYNMTFHEVFQQNPAVCGDPDEDGNVWPSYKKMANKTWRKALIDQNPAIAEAPAAAITTNNGLFLSNGQKAWKTGMHNLPANKADRKDFRFYSLRKPRRSFAVQIRPRCIIPSDTNQKVARIKLPKIDGAIKARGFNRKIWFGPDGKHTYEEALAAHELSNNLTVRVSKDTCGDYFICITFSQGKVKGDKPTWEFYQEVRVSPIPEPIGLDVGIKDIAILNTGTKYENKQFKRDRAATLKKMSRQLSRRWGPANSAFRDYNKNIRAENRALERAQQDPGSSGVGPEAPVLKSVAQPSRRYLTIQKNRAKLERKIARRRDTYYHQVTREVAGKSSLLAVETLRVKNMLQNHRLAFALSDAAMSDFISKLKYKARRIQVPLVSIGTFQPSSQTCSVCGSINPAVKNLSIRVWTCPNCGTRHNRDINAAKNILAIAQNMLEKKVPFADEGLPDEKPPAAPVKKAARKPRDAVFPDHPDLVIRFSKELTQLNDPRYVIVNKATNQIVDNAQGAGYRSAAKAKNCYKAKLAWSSKTNK

SEQ ID NO: 87 - protein, 575 aa, synthetic construct
MSVSFSLNAKKIRLENYAMKMRLYPSPTQAEQMDKMFLALRLAYNMTFHEVFQQNPAVCGDPDEDGNVWPSYKKMANKTWRKALIDQNPAIAEAPAAAITTNNGLFLSNGQKAWKTGMHNLPANKADRKDFRFYSLRKPRRSFAVQIRPRCIIPSDTNQKVARIKLPKIDGAIKARGFNRKIWFGPDGKHTYEEALAAHELSNNLTVRVSKDTCGDYFICITFSQGKVKGDKPTWEFYQEVRVSPIPEPIGLDVGIKDIAILNTGTKYENKQFKRDRAATLKKMSRQLSRRWGPANSAFRDYNKNIRAENRALERAQQDPGSSGVGPEAPVLKSVAQPSRRYLTIQKNRAKLERKIARRRDTYYHQVTREVAGKSSLLAVETLRVKNMLQNHRLAFALSDAAMSDFISKLKYKARRIQVPLVAIGTFQPSSQTCSVCGSINPAVKNLSIRVWTCPNCGTRHNRDINAAKNILAIAQNMLEKKVPFADEALPDEKPGAAPVKKAARKPRDRVFPDHPDLVIRFSKELTQLNDPRYVIVNKATNQIVDNAQGAGYRSAAKAKNCYKAKLAWSSKTNK

SEQ ID NO: 88 - DNA, 27 bp, synthetic construct
  source 1..27: mol_type = other DNA
aaacacagtaggagggacttacgttag

SEQ ID NO: 89 - DNA, 27 bp, synthetic construct
  source 1..27: mol_type = other DNA
cgagcgccgagtcgccactgcggcccc

SEQ ID NO: 90 - DNA, 27 bp, synthetic construct
  source 1..27: mol_type = other DNA
ccaggctcaaagtgatttaggggtggt

SEQ ID NO: 91 - DNA, 27 bp, synthetic construct
  source 1..27: mol_type = other DNA
ctagacaggggctagtatgtgcagctc

SEQ ID NO: 92 - DNA, 27 bp, synthetic construct
  source 1..27: mol_type = other DNA
ctgttgttgtttgtacttcctgatgca

SEQ ID NO: 93 - DNA, 27 bp, synthetic construct
  source 1..27: mol_type = other DNA
agcaccaggggcttcccttcctactcc

SEQ ID NO: 94 - DNA, 27 bp, synthetic construct
  source 1..27: mol_type = other DNA
ctctggggtacaaaacttttggtgaag

SEQ ID NO: 95 - DNA, 27 bp, synthetic construct
  source 1..27: mol_type = other DNA
agcaccaggggcttcccttcctactcc

SEQ ID NO: 96 - DNA, 27 bp, synthetic construct
  source 1..27: mol_type = other DNA
ttgtacctcaagagtggaaagaaatat

SEQ ID NO: 97 - DNA, 27 bp, synthetic construct
  source 1..27: mol_type = other DNA
agaaacagtgaacaacccactaaacca